European Patent Specification EP 3 765 048 B1, published August 27, 2025. Title: USING INFECTIOUS NUCLEIC ACID TO TREAT CANCER. Applicant: Mayo Foundation for Medical Education and Research. The sequence listing filed with the application follows.

SEQUENCE LISTING (69 sequences)

SEQ ID NO: 1 - DNA, 50 bp, artificial
  muscle-detargeting response element
acagctggttgaaggggaccaactggagccacacacttccttacattcca

SEQ ID NO: 2 - DNA, 102 bp, artificial
  muscle-detargeting response element
acagctggttgaaggggaccaacgatacagctggttgaaggggaccaactggagccacacacttccttacattccatcacccacacacttccttacattcca

SEQ ID NO: 3 - RNA, 100 nt, artificial
  coxsackievirus 3' UTR
cgacucauuuuaguaacccuaccucagucggauuggauuggguuauacuguuguagggguaaauuuuucuuuaauucggagaaaaaaaaaaaaaaaaaaa

SEQ ID NO: 4 - RNA, 123 nt, artificial
  coxsackievirus 3' terminal repeat
cgacucauuuuaguaaggcgcgccgacucauuuuaguaacccuaccucagucggauuggauuggguuauacuguuguagggguaaauuuuucuuuaauucggagaaaaaaaaaaaaaaaaaaa

SEQ ID NO: 5 - DNA, 10477 bp, artificial
  DNA encoding infectious nucleic acid
ttaaaacagctctggggttgttcccaccccagaggcccacgtggcggctagtactctggtattacggtacctttgtacgcctgttttgtatcccttcccccgtaactttagaagcttatcaaaagttcaatagcaggggtacaaaccagtacctctacgaacaagcacttctgtttccccggtgatatcacatagactgtacccacggtcaaaagtgattgatccgttatccgcttgagtacttcgagaagcctagtatcaccttggaatcttcgatgcgttgcgctcaacactctgccccgagtgtagcttaggctgatgagtctgggcactccccaccggcgacggtggcccaggctgcgttggcggcctacccatggctgatgccgtgggacgctagttgtgaacaaggtgtgaagagcctattgagctactcaagagtcctccggcccctgaatgcggctaatcctaaccacggagcaaccgctcacaacccagtgagtaggttgtcgtaatgcgtaagtctgtggcggaaccgactactttgggtgtccgtgtttccctttatattcatactggctgcttatggtgacaatttacaaattgttaccatatagctattggattggccacccagtattgtgcaatatatttgagtgtttctttcataagccttattaacatcacatttttaatcacaataaacagtgcaaatgggggctcaagtttcaacgcaaaagaccggtgcgcacgagaatcaaaacgtggcagccaatggatccaccattaattacactactatcaactattacaaagacagtgcgagtaattccgctactagacaagacctctcccaagatccatcaaaattcacagaaccggttaaggacttaatgttgaaaacagcaccagctctaaactcgcctaacgtggaagcatgtgggtacagtgaccgtgtgaggcaaatcactttaggcaactcgactattactacacaagaagcagccaatgctattgttgcttacggtgaatggcccacttacataaatgattcagaagctaatccggtagatgcacccactgagccagacgttagtagcaaccggttttacaccctagaatcggtgtcttggaagaccacttcaaggggatggtggtggaagttaccagattgtttgaaggacatgggaatgtttggtcagaatatgtactatcactacttggggcgctctggttacaccattcatgtccagtgcaacgcttcaaaatttcaccaaggggcgttaggagttttcctgataccagagtttgtcatggcttgcaacactgagagtaaaacgtcatacgtttcatacatcaatgcaaatcctggtgagagaggcggtgagtttacgaacacctacaatccgtcaaatacagacgccagtgagggcagaaagtttgcagcattggattatttgctgggttctggtgttctagcaggaaacgcctttgtgtacccgcaccagatcatcaacctacgtaccaacaacagtgcaacaattgtggtgccatacgtaaactcacttgtgattgattgtatggcaaaacacaataactggggcattgtcatattaccactggcacccttggcctttgccgcaacatcgtcaccacaggtgcctattacagtgaccattgcacccatgtgtacagaattcaatgggttgagaaacatcaccgtcccagtacatcaagggttgccgacaatgaacacacctggttccaatcaattccttacatctgatgacttccagtcgccctgtgccttacctaattttgatgttactccaccaatacacatacccggggaagtaaagaatatgatggaactagctgaaattgacacattgatcccaatgaacgcagtggacgggaaggtgaacacaatggagatgtatcaaataccattgaatgacaatttgagcaaggcacctatattctgtttatccctatcacctgcttctgataaacgactgagccacaccatgttgggtgaaatcctaaattattacacccattggacggggtccatcaggttcacctttctattttgtggcagtatgatggccactggtaaactgctcctcagctattccccaccgggagctaaaccaccaaccaatcgcaaggatgcaatgctaggcacacacatcatctgggacctagggttacaatccagttgttccatggttgcaccgtggatctccaacacagtgtacagacggtgtgcacgtgatgacttcactgagggcggatttataacttgcttctatcaaactagaattgtggtacctgcttcaacccctaccagtatgttcatgttaggctttgttagtgcgtgtccagacttcagtgtcagactgcttagggacactccccatattagtcaatcgaaactaataggacgtacacaaggcattgaagacctcattgacacagcgataaagaatgccttaagagtgtcccaaccaccctcgacccagtcaactgaagcaactagtggagtgaatagccaggaggtgccagctctaactgctgtggaaacaggagcatctggtcaagcaatccccagtgatgtggtggaaactaggcacgtggtaaattacaaaaccaggtctgaatcgtgtcttgagtcattctttgggagagctgcgtgtgtcacaatcctatccttgaccaactcctccaagagcggagaggagaaaaagcatttcaacatatggaatattacatacaccgacactgtccagttacgcagaaaattagaatttttcacgtattccaggtttgatcttgaaatgacttttgtattcacagagaactatcctagtacagccagtggagaagtgcgaaaccaggtgtaccagatcatgtatattccaccaggggcaccccgcccatcatcctgggatgactacacatggcaatcctcttcaaacccttccatcttctacatgtatggaaatgcacctccacggatgtcaattccttacgtagggattgccaatgcctattcacacttctacgatggctttgcacgggtgccacttgagggtgagaacaccgatgctggcgacacgttttacggtttagtgtccataaatgattttggagttttagcagttagagcagtaaaccgcagtaatccacatacaatacacacatctgtgagagtgtacatgaaaccaaaacacattcggtgttggtgccccagacctcctcgagctgtattatacaggggagagggagtggacatgatatccagtgcaattctacctctggccaaggtagactcaattaccacttttgggtttggtcatcagaacaaagcagtgtacgttgccggttacaagatttgcaactaccacctagcaaccccaagtgatcacttgaatgcaattagtatgttatgggacagggatttaatggtggtggaatctagagcccggggaactgataccatcgccagatgtagttgcaggtgtggagtttactattgtgaatctaggaggaagtactaccctgtcacttttactggcccaacgtttcgattcatggaagcaaacgactactatccagcaagataccagtctcacatgctgatagggtgcggatttgcagaacccggggactgcggtgggatactgaggtgcactcatggggtaattggtatcattactgcaggaggtgaaggggtagtagcctttgctgacattagagacctctgggtgtatgaagaggaggccatggaacagggaataacaagctacatcgaatctctcggcacagcctttggcgcagggttcacccacacaatcagtgagaaagtgactgaattgacaacgatggttaccagcactatcacagaaaaactactgaaaaacttggtgaaaatagtgtcggctctagtgattgttgtgagaaattatgaggacactaccacgatccttgcaacactagcactactcgggtgtgatatatctccttggcaatggttgaagaagaaggcatgtgacttactagagattccttatgtgatgcgccaaggtgatgggtggatgaagaaattcacagaggcgtgcaatgcagctaaaggcttagagtggattagcaacaaaatttccaagtttatagattggttgaagtgtaaaattatcccagacgctaaggacaaggtggaatttctcaccaagttgaaacagctagacatgttggaaaatcaaattgcaaccatccaccaatcttgccccagccaagaacaacaagagattcttttcaacaatgtgagatggttagcagtccagtcccgtcggtttgcaccattatacgctgtggaggcacgccgaattaacaaaatggagagcacaataaacaattatatacagttcaagagcaaacaccgtattgaaccagtatgtatgctcattcatgggtcaccagggacgggtaaatctatagctacttcattaataggtagagcaatagcagagaaggaaagcacatcagtctattcaatgccacctgacccatctcactttgatggctataaacaacaaggggtagtgattatggacgacctaaaccaaaaccccgatggtatggacatgaaactgttttgccaaatggtatcaacagtggagtttattcctccaatggcctcattagaggagaagggcattttgtttacatctgattatgtcctggcttctaccaactctcattcaattgtaccacccacagtggctcacagtgatgccttaaccagacgatttgcatttgatgtggaggtttacacgatgtctgaacattcagtcaaaggcaaactgaatatggccacggccactcaattgtgtaaggattgtccaacacctgcaaattttaaaaagtgttgccctctcgtttgtggaaaggccttgcaattaatggacaggtacaccagacaaaggttcactgtagatgagattaccacattaatcatgaatgagaaaaacagaagggccaatatcggcaattgcatggaagccttgtttcaaggaccactaaggtataaagatttgaagatcgatgtgaagacagttcccccccctgagtgcatcagtgatttgttacaagcagtggattctcaagaggttagggattactgtgagaagaaaggctggatcgttaacgttactagccagattcaactagaaaggaacatcaatagggccatgactatactccaagctgttaccacattcgcagcagtcgcaggagtagtgtatgtaatgtacaaactcttcgccggtcaacagggtgcatacactggcttgccaaacaaaaaacccaatgtccctactatcagagtcgctaaagtccaggggccaggatttgactacgcagtggcaatggcaaaaagaaacatagttactgcaaccaccaccaagggtgaatttaccatgctaggggtgcatgataatgtagcaatattgccaacccatgccgctccaggagaaaccattattattgatgggaaagaagtagagatcctagacgccagagccttagaagatcaagcgggaaccaatcttgagatcaccattattactctaaaaagaaatgagaagtttagagacatcagatcacatattcccacccaaattactgaaactaacgatggagtgttgatcgtgaacactagcaagtaccccaatatgtatgtccccgttggtgctgtgaccgaacagggatatcttaatctcagtggacgtcaaactgctcgcactttaatgtacaactttccaacaagggcaggccagtgcggaggaatcatcacttgtactggcaaagtcattgggatgcatgttggcgggaacggttcacatgggtttgctgcagccctcaagcgatcatacttcactcaaaatcagggcgaaatccagtggatgaggtcatcaaaagaagtggggtaccccattataaatgccccatccaagacaaagttagaacccagtgctttccactatgtttttgaaggtgttaaggaaccagctgtactcactaagaatgaccccagactaaaaacagattttgaagaagccatcttttctaaatatgtggggaacaaaattactgaagtggacgagtacatgaaagaagcagtggatcactatgcaggacagttaatgtcactggatatcaacacagaacagatgtgcctggaggatgccatgtacggtaccgatggtcttgaggccctggatcttagcactagtgctggatatccttatgttgcaatggggaaaaagaaaagagacattctagataaacagaccagagatactaaggagatgcagagacttttagatacctatggaatcaatctaccattagtcacgtacgtgaaagatgaactcaggtcaaagactaaagtggaacaaggaaagtcaagattgattgaagcttccagccttaatgattcagttgcaatgagaatggcctttggcaatctttacgcagctttccacaagaatccaggtgtggtgacaggatcagcagttggttgtgacccagatttgttttggagtaagataccagtgctaatggaagaaaaactcttcgcttttgactacacagggtatgatgcctcactcagccctgcttggtttgaagctcttaaaatggtgttagaaaaaattggatttggcagtagagtagactatatagactacctgaaccactctcaccacctttacaaaaacaagacttattgtgtcaaaggcggcatgccatccggctgctctggcacctcaattttcaactcaatgattaacaacctgatcattaggacgcttttactgagaacctacaagggcatagacttggaccatttaaaaatgattgcctatggtgatgacgtgatagcttcctacccccatgaggttgacgctagtctcctagcccaatcaggaaaagactatggactaaccatgactccagcagataaatcagcaacctttgaaacagtcacatgggagaatgtaacatttctgaaaagatttttcagagcagatgagaagtatccattcctggtgcatccagtgatgccaatgaaagaaattcacgaatcaatcagatggaccaaggaccctagaaacacacaggatcacgtacgctcgttgtgcctattagcttggcacaacggtgaagaagaatacaataaatttttagctaaaatcagaagtgtgccaatcggaagagctttattgctcccagagtactctacattgtaccgccgatggctcgactcattttagtaaccctacctcagtcggattggattgggttatactgttgtaggggtaaatttttctttaattcggagaaaaaaaaaaaaaaaaaaagagctcccaatcactagtgaattcgcggccgcctgcaggtcgaccatatgggagagctcccaacgcgttggatgcatagcttgagtattctatagtgtcacctaaatagcttggcgtaatcatggtcatagctgtttcctgtgtgaaattgttatccgctcacaattccacacaacatacgagccggaagcataaagtgtaaagcctggggtgcctaatgagtgagctaactcacattaattgcgttgcgctcactgcccgctttccagtcgggaaacctgtcgtgccagctgcattaatgaatcggccaacgcgcggggagaggcggtttgcgtattgggcgctcttccgcttcctcgctcactgactcgctgcgctcggtcgttcggctgcggcgagcggtatcagctcactcaaaggcggtaatacggttatccacagaatcaggggataacgcaggaaagaacatgtgagcaaaaggccagcaaaaggccaggaaccgtaaaaaggccgcgttgctggcgtttttccataggctccgcccccctgacgagcatcacaaaaatcgacgctcaagtcagaggtggcgaaacccgacaggactataaagataccaggcgtttccccctggaagctccctcgtgcgctctcctgttccgaccctgccgcttaccggatacctgtccgcctttctcccttcgggaagcgtggcgctttctcatagctcacgctgtaggtatctcagttcggtgtaggtcgttcgctccaagctgggctgtgtgcacgaaccccccgttcagcccgaccgctgcgccttatccggtaactatcgtcttgagtccaacccggtaagacacgacttatcgccactggcagcagccactggtaacaggattagcagagcgaggtatgtaggcggtgctacagagttcttgaagtggtggcctaactacggctacactagaagaacagtatttggtatctgcgctctgctgaagccagttaccttcggaaaaagagttggtagctcttgatccggcaaacaaaccaccgctggtagcggtggtttttttgtttgcaagcagcagattacgcgcagaaaaaaaggatctcaagaagatcctttgatcttttctacggggtctgacgctcagtggaacgaaaactcacgttaagggattttggtcatgagattatcaaaaaggatcttcacctagatccttttaaattaaaaatgaagttttaaatcaatctaaagtatatatgagtaaacttggtctgacagttaccaatgcttaatcagtgaggcacctatctcagcgatctgtctatttcgttcatccatagttgcctgactccccgtcgtgtagataactacgatacgggagggcttaccatctggccccagtgctgcaatgataccgcgagacccacgctcaccggctccagatttatcagcaataaaccagccagccggaagggccgagcgcagaagtggtcctgcaactttatccgcctccatccagtctattaattgttgccgggaagctagagtaagtagttcgccagttaatagtttgcgcaacgttgttgccattgctacaggcatcgtggtgtcacgctcgtcgtttggtatggcttcattcagctccggttcccaacgatcaaggcgagttacatgatcccccatgttgtgcaaaaaagcggttagctccttcggtcctccgatcgttgtcagaagtaagttggccgcagtgttatcactcatggttatggcagcactgcataattctcttactgtcatgccatccgtaagatgcttttctgtgactggtgagtactcaaccaagtcattctgagaatagtgtatgcggcgaccgagttgctcttgcccggcgtcaatacgggataataccgcgccacatagcagaactttaaaagtgctcatcattggaaaacgttcttcggggcgaaaactctcaaggatcttaccgctgttgagatccagttcgatgtaacccactcgtgcacccaactgatcttcagcatcttttactttcaccagcgtttctgggtgagcaaaaacaggaaggcaaaatgccgcaaaaaagggaataagggcgacacggaaatgttgaatactcatactcttcctttttcaatattattgaagcatttatcagggttattgtctcatgagcggatacatatttgaatgtatttagaaaaataaacaaataggggttccgcgcacatttccccgaaaagtgccacctgatgcggtgtgaaataccgcacagatgcgtaaggagaaaataccgcatcaggaaattgtaagcgttaatattttgttaaaattcgcgttaaatttttgttaaatcagctcattttttaaccaataggccgaaatcggcaaaatcccttataaatcaaaagaatagaccgagatagggttgagtgttgttccagtttggaacaagagtccactattaaagaacgtggactccaacgtcaaagggcgaaaaaccgtctatcagggcgatggcccactacgtgaaccatcaccctaatcaagttttttggggtcgaggtgccgtaaagcactaaatcggaaccctaaagggagcccccgatttagagcttgacggggaaagccggcgaacgtggcgagaaaggaagggaagaaagcgaaaggagcgggcgctagggcgctggcaagtgtagcggtcacgctgcgcgtaaccaccacacccgccgcgcttaatgcgccgctacagggcgcgtccattcgccattcaggctgcgcaactgttgggaagggcgatcggtgcgggcctcttcgctattacgccagctggcgaaagggggatgtgctgcaaggcgattaagttgggtaacgccagggttttcccagtcacgacgttgtaaaacgacggccagtgaattgtaatacgactcactatagggcgaattgggcccgacgtcgcatgctcccggccgccatggcggccgcgggaattcgattgaggcatgctaatacgactcactatagg

SEQ ID NO: 6 - DNA, 10474 bp, artificial
  DNA encoding infectious nucleic acid
ttaaaacagctctggggttgttcccaccccagaggcccacgtggcggctagtactctggtattacggtacctttgtacgcctgttttgtatcccttcccccgtaactttagaagcttatcaaaagttcaatagcaggggtacaaaccagtacctctacgaacaagcacttctgtttccccggtgatatcacatagactgtacccacggtcaaaagtgattgatccgttatccgcttgagtacttcgagaagcctagtatcaccttggaatcttcgatgcgttgcgctcaacactctgccccgagtgtagcttaggctgatgagtctgggcactccccaccggcgacggtggcccaggctgcgttggcggcctacccatggctgatgccgtgggacgctagttgtgaacaaggtgtgaagagcctattgagctactcaagagtcctccggcccctgaatgcggctaatcctaaccacggagcaaccgctcacaacccagtgagtaggttgtcgtaatgcgtaagtctgtggcggaaccgactactttgggtgtccgtgtttccctttatattcatactggctgcttatggtgacaatttacaaattgttaccatatagctattggattggcgcgccgcacagctggttgaaggggaccaactggagccacacacttccttacattccacggcgcgccaataaacagtgcaaatgggggctcaagtttcaacgcaaaagaccggtgcgcacgagaatcaaaacgtggcagccaatggatccaccattaattacactactatcaactattacaaagacagtgcgagtaattccgctactagacaagacctctcccaagatccatcaaaattcacagaaccggttaaggacttaatgttgaaaacagcaccagctctaaactcgcctaacgtggaagcatgtgggtacagtgaccgtgtgaggcaaatcactttaggcaactcgactattactacacaagaagcagccaatgctattgttgcttacggtgaatggcccacttacataaatgattcagaagctaatccggtagatgcacccactgagccagacgttagtagcaaccggttttacaccctagaatcggtgtcttggaagaccacttcaaggggatggtggtggaagttaccagattgtttgaaggacatgggaatgtttggtcagaatatgtactatcactacttggggcgctctggttacaccattcatgtccagtgcaacgcttcaaaatttcaccaaggggcgttaggagttttcctgataccagagtttgtcatggcttgcaacactgagagtaaaacgtcatacgtttcatacatcaatgcaaatcctggtgagagaggcggtgagtttacgaacacctacaatccgtcaaatacagacgccagtgagggcagaaagtttgcagcattggattatttgctgggttctggtgttctagcaggaaacgcctttgtgtacccgcaccagatcatcaacctacgtaccaacaacagtgcaacaattgtggtgccatacgtaaactcacttgtgattgattgtatggcaaaacacaataactggggcattgtcatattaccactggcacccttggcctttgccgcaacatcgtcaccacaggtgcctattacagtgaccattgcacccatgtgtacagaattcaatgggttgagaaacatcaccgtcccagtacatcaagggttgccgacaatgaacacacctggttccaatcaattccttacatctgatgacttccagtcgccctgtgccttacctaattttgatgttactccaccaatacacatacccggggaagtaaagaatatgatggaactagctgaaattgacacattgatcccaatgaacgcagtggacgggaaggtgaacacaatggagatgtatcaaataccattgaatgacaatttgagcaaggcacctatattctgtttatccctatcacctgcttctgataaacgactgagccacaccatgttgggtgaaatcctaaattattacacccattggacggggtccatcaggttcacctttctattttgtggcagtatgatggccactggtaaactgctcctcagctattccccaccgggagctaaaccaccaaccaatcgcaaggatgcaatgctaggcacacacatcatctgggacctagggttacaatccagttgttccatggttgcaccgtggatctccaacacagtgtacagacggtgtgcacgtgatgacttcactgagggcggatttataacttgcttctatcaaactagaattgtggtacctgcttcaacccctaccagtatgttcatgttaggctttgttagtgcgtgtccagacttcagtgtcagactgcttagggacactccccatattagtcaatcgaaactaataggacgtacacaaggcattgaagacctcattgacacagcgataaagaatgccttaagagtgtcccaaccaccctcgacccagtcaactgaagcaactagtggagtgaatagccaggaggtgccagctctaactgctgtggaaacaggagcatctggtcaagcaatccccagtgatgtggtggaaactaggcacgtggtaaattacaaaaccaggtctgaatcgtgtcttgagtcattctttgggagagctgcgtgtgtcacaatcctatccttgaccaactcctccaagagcggagaggagaaaaagcatttcaacatatggaatattacatacaccgacactgtccagttacgcagaaaattagaatttttcacgtattccaggtttgatcttgaaatgacttttgtattcacagagaactatcctagtacagccagtggagaagtgcgaaaccaggtgtaccagatcatgtatattccaccaggggcaccccgcccatcatcctgggatgactacacatggcaatcctcttcaaacccttccatcttctacatgtatggaaatgcacctccacggatgtcaattccttacgtagggattgccaatgcctattcacacttctacgatggctttgcacgggtgccacttgagggtgagaacaccgatgctggcgacacgttttacggtttagtgtccataaatgattttggagttttagcagttagagcagtaaaccgcagtaatccacatacaatacacacatctgtgagagtgtacatgaaaccaaaacacattcggtgttggtgccccagacctcctcgagctgtattatacaggggagagggagtggacatgatatccagtgcaattctacctctggccaaggtagactcaattaccacttttgggtttggtcatcagaacaaagcagtgtacgttgccggttacaagatttgcaactaccacctagcaaccccaagtgatcacttgaatgcaattagtatgttatgggacagggatttaatggtggtggaatctagagcccggggaactgataccatcgccagatgtagttgcaggtgtggagtttactattgtgaatctaggaggaagtactaccctgtcacttttactggcccaacgtttcgattcatggaagcaaacgactactatccagcaagataccagtctcacatgctgatagggtgcggatttgcagaacccggggactgcggtgggatactgaggtgcactcatggggtaattggtatcattactgcaggaggtgaaggggtagtagcctttgctgacattagagacctctgggtgtatgaagaggaggccatggaacagggaataacaagctacatcgaatctctcggcacagcctttggcgcagggttcacccacacaatcagtgagaaagtgactgaattgacaacgatggttaccagcactatcacagaaaaactactgaaaaacttggtgaaaatagtgtcggctctagtgattgttgtgagaaattatgaggacactaccacgatccttgcaacactagcactactcgggtgtgatatatctccttggcaatggttgaagaagaaggcatgtgacttactagagattccttatgtgatgcgccaaggtgatgggtggatgaagaaattcacagaggcgtgcaatgcagctaaaggcttagagtggattagcaacaaaatttccaagtttatagattggttgaagtgtaaaattatcccagacgctaaggacaaggtggaatttctcaccaagttgaaacagctagacatgttggaaaatcaaattgcaaccatccaccaatcttgccccagccaagaacaacaagagattcttttcaacaatgtgagatggttagcagtccagtcccgtcggtttgcaccattatacgctgtggaggcacgccgaattaacaaaatggagagcacaataaacaattatatacagttcaagagcaaacaccgtattgaaccagtatgtatgctcattcatgggtcaccagggacgggtaaatctatagctacttcattaataggtagagcaatagcagagaaggaaagcacatcagtctattcaatgccacctgacccatctcactttgatggctataaacaacaaggggtagtgattatggacgacctaaaccaaaaccccgatggtatggacatgaaactgttttgccaaatggtatcaacagtggagtttattcctccaatggcctcattagaggagaagggcattttgtttacatctgattatgtcctggcttctaccaactctcattcaattgtaccacccacagtggctcacagtgatgccttaaccagacgatttgcatttgatgtggaggtttacacgatgtctgaacattcagtcaaaggcaaactgaatatggccacggccactcaattgtgtaaggattgtccaacacctgcaaattttaaaaagtgttgccctctcgtttgtggaaaggccttgcaattaatggacaggtacaccagacaaaggttcactgtagatgagattaccacattaatcatgaatgagaaaaacagaagggccaatatcggcaattgcatggaagccttgtttcaaggaccactaaggtataaagatttgaagatcgatgtgaagacagttcccccccctgagtgcatcagtgatttgttacaagcagtggattctcaagaggttagggattactgtgagaagaaaggctggatcgttaacgttactagccagattcaactagaaaggaacatcaatagggccatgactatactccaagctgttaccacattcgcagcagtcgcaggagtagtgtatgtaatgtacaaactcttcgccggtcaacagggtgcatacactggcttgccaaacaaaaaacccaatgtccctactatcagagtcgctaaagtccaggggccaggatttgactacgcagtggcaatggcaaaaagaaacatagttactgcaaccaccaccaagggtgaatttaccatgctaggggtgcatgataatgtagcaatattgccaacccatgccgctccaggagaaaccattattattgatgggaaagaagtagagatcctagacgccagagccttagaagatcaagcgggaaccaatcttgagatcaccattattactctaaaaagaaatgagaagtttagagacatcagatcacatattcccacccaaattactgaaactaacgatggagtgttgatcgtgaacactagcaagtaccccaatatgtatgtccccgttggtgctgtgaccgaacagggatatcttaatctcagtggacgtcaaactgctcgcactttaatgtacaactttccaacaagggcaggccagtgcggaggaatcatcacttgtactggcaaagtcattgggatgcatgttggcgggaacggttcacatgggtttgctgcagccctcaagcgatcatacttcactcaaaatcagggcgaaatccagtggatgaggtcatcaaaagaagtggggtaccccattataaatgccccatccaagacaaagttagaacccagtgctttccactatgtttttgaaggtgttaaggaaccagctgtactcactaagaatgaccccagactaaaaacagattttgaagaagccatcttttctaaatatgtggggaacaaaattactgaagtggacgagtacatgaaagaagcagtggatcactatgcaggacagttaatgtcactggatatcaacacagaacagatgtgcctggaggatgccatgtacggtaccgatggtcttgaggccctggatcttagcactagtgctggatatccttatgttgcaatggggaaaaagaaaagagacattctagataaacagaccagagatactaaggagatgcagagacttttagatacctatggaatcaatctaccattagtcacgtacgtgaaagatgaactcaggtcaaagactaaagtggaacaaggaaagtcaagattgattgaagcttccagccttaatgattcagttgcaatgagaatggcctttggcaatctttacgcagctttccacaagaatccaggtgtggtgacaggatcagcagttggttgtgacccagatttgttttggagtaagataccagtgctaatggaagaaaaactcttcgcttttgactacacagggtatgatgcctcactcagccctgcttggtttgaagctcttaaaatggtgttagaaaaaattggatttggcagtagagtagactatatagactacctgaaccactctcaccacctttacaaaaacaagacttattgtgtcaaaggcggcatgccatccggctgctctggcacctcaattttcaactcaatgattaacaacctgatcattaggacgcttttactgagaacctacaagggcatagacttggaccatttaaaaatgattgcctatggtgatgacgtgatagcttcctacccccatgaggttgacgctagtctcctagcccaatcaggaaaagactatggactaaccatgactccagcagataaatcagcaacctttgaaacagtcacatgggagaatgtaacatttctgaaaagatttttcagagcagatgagaagtatccattcctggtgcatccagtgatgccaatgaaagaaattcacgaatcaatcagatggaccaaggaccctagaaacacacaggatcacgtacgctcgttgtgcctattagcttggcacaacggtgaagaagaatacaataaatttttagctaaaatcagaagtgtgccaatcggaagagctttattgctcccagagtactctacattgtaccgccgatggctcgactcattttagtaaccctacctcagtcggattggattgggttatactgttgtaggggtaaatttttctttaattcggagaaaaaaaaaaaaaaaaaaagagctcccaatcactagtgaattcgcggccgcctgcaggtcgaccatatgggagagctcccaacgcgttggatgcatagcttgagtattctatagtgtcacctaaatagcttggcgtaatcatggtcatagctgtttcctgtgtgaaattgttatccgctcacaattccacacaacatacgagccggaagcataaagtgtaaagcctggggtgcctaatgagtgagctaactcacattaattgcgttgcgctcactgcccgctttccagtcgggaaacctgtcgtgccagctgcattaatgaatcggccaacgcgcggggagaggcggtttgcgtattgggcgctcttccgcttcctcgctcactgactcgctgcgctcggtcgttcggctgcggcgagcggtatcagctcactcaaaggcggtaatacggttatccacagaatcaggggataacgcaggaaagaacatgtgagcaaaaggccagcaaaaggccaggaaccgtaaaaaggccgcgttgctggcgtttttccataggctccgcccccctgacgagcatcacaaaaatcgacgctcaagtcagaggtggcgaaacccgacaggactataaagataccaggcgtttccccctggaagctccctcgtgcgctctcctgttccgaccctgccgcttaccggatacctgtccgcctttctcccttcgggaagcgtggcgctttctcatagctcacgctgtaggtatctcagttcggtgtaggtcgttcgctccaagctgggctgtgtgcacgaaccccccgttcagcccgaccgctgcgccttatccggtaactatcgtcttgagtccaacccggtaagacacgacttatcgccactggcagcagccactggtaacaggattagcagagcgaggtatgtaggcggtgctacagagttcttgaagtggtggcctaactacggctacactagaagaacagtatttggtatctgcgctctgctgaagccagttaccttcggaaaaagagttggtagctcttgatccggcaaacaaaccaccgctggtagcggtggtttttttgtttgcaagcagcagattacgcgcagaaaaaaaggatctcaagaagatcctttgatcttttctacggggtctgacgctcagtggaacgaaaactcacgttaagggattttggtcatgagattatcaaaaaggatcttcacctagatccttttaaattaaaaatgaagttttaaatcaatctaaagtatatatgagtaaacttggtctgacagttaccaatgcttaatcagtgaggcacctatctcagcgatctgtctatttcgttcatccatagttgcctgactccccgtcgtgtagataactacgatacgggagggcttaccatctggccccagtgctgcaatgataccgcgagacccacgctcaccggctccagatttatcagcaataaaccagccagccggaagggccgagcgcagaagtggtcctgcaactttatccgcctccatccagtctattaattgttgccgggaagctagagtaagtagttcgccagttaatagtttgcgcaacgttgttgccattgctacaggcatcgtggtgtcacgctcgtcgtttggtatggcttcattcagctccggttcccaacgatcaaggcgagttacatgatcccccatgttgtgcaaaaaagcggttagctccttcggtcctccgatcgttgtcagaagtaagttggccgcagtgttatcactcatggttatggcagcactgcataattctcttactgtcatgccatccgtaagatgcttttctgtgactggtgagtactcaaccaagtcattctgagaatagtgtatgcggcgaccgagttgctcttgcccggcgtcaatacgggataataccgcgccacatagcagaactttaaaagtgctcatcattggaaaacgttcttcggggcgaaaactctcaaggatcttaccgctgttgagatccagttcgatgtaacccactcgtgcacccaactgatcttcagcatcttttactttcaccagcgtttctgggtgagcaaaaacaggaaggcaaaatgccgcaaaaaagggaataagggcgacacggaaatgttgaatactcatactcttcctttttcaatattattgaagcatttatcagggttattgtctcatgagcggatacatatttgaatgtatttagaaaaataaacaaataggggttccgcgcacatttccccgaaaagtgccacctgatgcggtgtgaaataccgcacagatgcgtaaggagaaaataccgcatcaggaaattgtaagcgttaatattttgttaaaattcgcgttaaatttttgttaaatcagctcattttttaaccaataggccgaaatcggcaaaatcccttataaatcaaaagaatagaccgagatagggttgagtgttgttccagtttggaacaagagtccactattaaagaacgtggactccaacgtcaaagggcgaaaaaccgtctatcagggcgatggcccactacgtgaaccatcaccctaatcaagttttttggggtcgaggtgccgtaaagcactaaatcggaaccctaaagggagcccccgatttagagcttgacggggaaagccggcgaacgtggcgagaaaggaagggaagaaagcgaaaggagcgggcgctagggcgctggcaagtgtagcggtcacgctgcgcgtaaccaccacacccgccgcgcttaatgcgccgctacagggcgcgtccattcgccattcaggctgcgcaactgttgggaagggcgatcggtgcgggcctcttcgctattacgccagctggcgaaagggggatgtgctgcaaggcgattaagttgggtaacgccagggttttcccagtcacgacgttgtaaaacgacggccagtgaattgtaatacgactcactatagggcgaattgggcccgacgtcgcatgctcccggccgccatggcggccgcgggaattcgattgaggcatgctaatacgactcactatagg

SEQ ID NO: 7 - DNA, 10526 bp, artificial
  DNA encoding infectious nucleic acid
ttaaaacagctctggggttgttcccaccccagaggcccacgtggcggctagtactctggtattacggtacctttgtacgcctgttttgtatcccttcccccgtaactttagaagcttatcaaaagttcaatagcaggggtacaaaccagtacctctacgaacaagcacttctgtttccccggtgatatcacatagactgtacccacggtcaaaagtgattgatccgttatccgcttgagtacttcgagaagcctagtatcaccttggaatcttcgatgcgttgcgctcaacactctgccccgagtgtagcttaggctgatgagtctgggcactccccaccggcgacggtggcccaggctgcgttggcggcctacccatggctgatgccgtgggacgctagttgtgaacaaggtgtgaagagcctattgagctactcaagagtcctccggcccctgaatgcggctaatcctaaccacggagcaaccgctcacaacccagtgagtaggttgtcgtaatgcgtaagtctgtggcggaaccgactactttgggtgtccgtgtttccctttatattcatactggctgcttatggtgacaatttacaaattgttaccatatagctattggattggcgcgccgcacagctggttgaaggggaccaacgatacagctggttgaaggggaccaactggagccacacacttccttacattccatcacccacacacttccttacattccacggcgcgccaataaacagtgcaaatgggggctcaagtttcaacgcaaaagaccggtgcgcacgagaatcaaaacgtggcagccaatggatccaccattaattacactactatcaactattacaaagacagtgcgagtaattccgctactagacaagacctctcccaagatccatcaaaattcacagaaccggttaaggacttaatgttgaaaacagcaccagctctaaactcgcctaacgtggaagcatgtgggtacagtgaccgtgtgaggcaaatcactttaggcaactcgactattactacacaagaagcagccaatgctattgttgcttacggtgaatggcccacttacataaatgattcagaagctaatccggtagatgcacccactgagccagacgttagtagcaaccggttttacaccctagaatcggtgtcttggaagaccacttcaaggggatggtggtggaagttaccagattgtttgaaggacatgggaatgtttggtcagaatatgtactatcactacttggggcgctctggttacaccattcatgtccagtgcaacgcttcaaaatttcaccaaggggcgttaggagttttcctgataccagagtttgtcatggcttgcaacactgagagtaaaacgtcatacgtttcatacatcaatgcaaatcctggtgagagaggcggtgagtttacgaacacctacaatccgtcaaatacagacgccagtgagggcagaaagtttgcagcattggattatttgctgggttctggtgttctagcaggaaacgcctttgtgtacccgcaccagatcatcaacctacgtaccaacaacagtgcaacaattgtggtgccatacgtaaactcacttgtgattgattgtatggcaaaacacaataactggggcattgtcatattaccactggcacccttggcctttgccgcaacatcgtcaccacaggtgcctattacagtgaccattgcacccatgtgtacagaattcaatgggttgagaaacatcaccgtcccagtacatcaagggttgccgacaatgaacacacctggttccaatcaattccttacatctgatgacttccagtcgccctgtgccttacctaattttgatgttactccaccaatacacatacccggggaagtaaagaatatgatggaactagctgaaattgacacattgatcccaatgaacgcagtggacgggaaggtgaacacaatggagatgtatcaaataccattgaatgacaatttgagcaaggcacctatattctgtttatccctatcacctgcttctgataaacgactgagccacaccatgttgggtgaaatcctaaattattacacccattggacggggtccatcaggttcacctttctattttgtggcagtatgatggccactggtaaactgctcctcagctattccccaccgggagctaaaccaccaaccaatcgcaaggatgcaatgctaggcacacacatcatctgggacctagggttacaatccagttgttccatggttgcaccgtggatctccaacacagtgtacagacggtgtgcacgtgatgacttcactgagggcggatttataacttgcttctatcaaactagaattgtggtacctgcttcaacccctaccagtatgttcatgttaggctttgttagtgcgtgtccagacttcagtgtcagactgcttagggacactccccatattagtcaatcgaaactaataggacgtacacaaggcattgaagacctcattgacacagcgataaagaatgccttaagagtgtcccaaccaccctcgacccagtcaactgaagcaactagtggagtgaatagccaggaggtgccagctctaactgctgtggaaacaggagcatctggtcaagcaatccccagtgatgtggtggaaactaggcacgtggtaaattacaaaaccaggtctgaatcgtgtcttgagtcattctttgggagagctgcgtgtgtcacaatcctatccttgaccaactcctccaagagcggagaggagaaaaagcatttcaacatatggaatattacatacaccgacactgtccagttacgcagaaaattagaatttttcacgtattccaggtttgatcttgaaatgacttttgtattcacagagaactatcctagtacagccagtggagaagtgcgaaaccaggtgtaccagatcatgtatattccaccaggggcaccccgcccatcatcctgggatgactacacatggcaatcctcttcaaacccttccatcttctacatgtatggaaatgcacctccacggatgtcaattccttacgtagggattgccaatgcctattcacacttctacgatggctttgcacgggtgccacttgagggtgagaacaccgatgctggcgacacgttttacggtttagtgtccataaatgattttggagttttagcagttagagcagtaaaccgcagtaatccacatacaatacacacatctgtgagagtgtacatgaaaccaaaacacattcggtgttggtgccccagacctcctcgagctgtattatacaggggagagggagtggacatgatatccagtgcaattctacctctggccaaggtagactcaattaccacttttgggtttggtcatcagaacaaagcagtgtacgttgccggttacaagatttgcaactaccacctagcaaccccaagtgatcacttgaatgcaattagtatgttatgggacagggatttaatggtggtggaatctagagcccggggaactgataccatcgccagatgtagttgcaggtgtggagtttactattgtgaatctaggaggaagtactaccctgtcacttttactggcccaacgtttcgattcatggaagcaaacgactactatccagcaagataccagtctcacatgctgatagggtgcggatttgcagaacccggggactgcggtgggatactgaggtgcactcatggggtaattggtatcattactgcaggaggtgaaggggtagtagcctttgctgacattagagacctctgggtgtatgaagaggaggccatggaacagggaataacaagctacatcgaatctctcggcacagcctttggcgcagggttcacccacacaatcagtgagaaagtgactgaattgacaacgatggttaccagcactatcacagaaaaactactgaaaaacttggtgaaaatagtgtcggctctagtgattgttgtgagaaattatgaggacactaccacgatccttgcaacactagcactactcgggtgtgatatatctccttggcaatggttgaagaagaaggcatgtgacttactagagattccttatgtgatgcgccaaggtgatgggtggatgaagaaattcacagaggcgtgcaatgcagctaaaggcttagagtggattagcaacaaaatttccaagtttatagattggttgaagtgtaaaattatcccagacgctaaggacaaggtggaatttctcaccaagttgaaacagctagacatgttggaaaatcaaattgcaaccatccaccaatcttgccccagccaagaacaacaagagattcttttcaacaatgtgagatggttagcagtccagtcccgtcggtttgcaccattatacgctgtggaggcacgccgaattaacaaaatggagagcacaataaacaattatatacagttcaagagcaaacaccgtattgaaccagtatgtatgctcattcatgggtcaccagggacgggtaaatctatagctacttcattaataggtagagcaatagcagagaaggaaagcacatcagtctattcaatgccacctgacccatctcactttgatggctataaacaacaaggggtagtgattatggacgacctaaaccaaaaccccgatggtatggacatgaaactgttttgccaaatggtatcaacagtggagtttattcctccaatggcctcattagaggagaagggcattttgtttacatctgattatgtcctggcttctaccaactctcattcaattgtaccacccacagtggctcacagtgatgccttaaccagacgatttgcatttgatgtggaggtttacacgatgtctgaacattcagtcaaaggcaaactgaatatggccacggccactcaattgtgtaaggattgtccaacacctgcaaattttaaaaagtgttgccctctcgtttgtggaaaggccttgcaattaatggacaggtacaccagacaaaggttcactgtagatgagattaccacattaatcatgaatgagaaaaacagaagggccaatatcggcaattgcatggaagccttgtttcaaggaccactaaggtataaagatttgaagatcgatgtgaagacagttcccccccctgagtgcatcagtgatttgttacaagcagtggattctcaagaggttagggattactgtgagaagaaaggctggatcgttaacgttactagccagattcaactagaaaggaacatcaatagggccatgactatactccaagctgttaccacattcgcagcagtcgcaggagtagtgtatgtaatgtacaaactcttcgccggtcaacagggtgcatacactggcttgccaaacaaaaaacccaatgtccctactatcagagtcgctaaagtccaggggccaggatttgactacgcagtggcaatggcaaaaagaaacatagttactgcaaccaccaccaagggtgaatttaccatgctaggggtgcatgataatgtagcaatattgccaacccatgccgctccaggagaaaccattattattgatgggaaagaagtagagatcctagacgccagagccttagaagatcaagcgggaaccaatcttgagatcaccattattactctaaaaagaaatgagaagtttagagacatcagatcacatattcccacccaaattactgaaactaacgatggagtgttgatcgtgaacactagcaagtaccccaatatgtatgtccccgttggtgctgtgaccgaacagggatatcttaatctcagtggacgtcaaactgctcgcactttaatgtacaactttccaacaagggcaggccagtgcggaggaatcatcacttgtactggcaaagtcattgggatgcatgttggcgggaacggttcacatgggtttgctgcagccctcaagcgatcatacttcactcaaaatcagggcgaaatccagtggatgaggtcatcaaaagaagtggggtaccccattataaatgccccatccaagacaaagttagaacccagtgctttccactatgtttttgaaggtgttaaggaaccagctgtactcactaagaatgaccccagactaaaaacagattttgaagaagccatcttttctaaatatgtggggaacaaaattactgaagtggacgagtacatgaaagaagcagtggatcactatgcaggacagttaatgtcactggatatcaacacagaacagatgtgcctggaggatgccatgtacggtaccgatggtcttgaggccctggatcttagcactagtgctggatatccttatgttgcaatggggaaaaagaaaagagacattctagataaacagaccagagatactaaggagatgcagagacttttagatacctatggaatcaatctaccattagtcacgtacgtgaaagatgaactcaggtcaaagactaaagtggaacaaggaaagtcaagattgattgaagcttccagccttaatgattcagttgcaatgagaatggcctttggcaatctttacgcagctttccacaagaatccaggtgtggtgacaggatcagcagttggttgtgacccagatttgttttggagtaagataccagtgctaatggaagaaaaactcttcgcttttgactacacagggtatgatgcctcactcagccctgcttggtttgaagctcttaaaatggtgttagaaaaaattggatttggcagtagagtagactatatagactacctgaaccactctcaccacctttacaaaaacaagacttattgtgtcaaaggcggcatgccatccggctgctctggcacctcaattttcaactcaatgattaacaacctgatcattaggacgcttttactgagaacctacaagggcatagacttggaccatttaaaaatgattgcctatggtgatgacgtgatagcttcctacccccatgaggttgacgctagtctcctagcccaatcaggaaaagactatggactaaccatgactccagcagataaatcagcaacctttgaaacagtcacatgggagaatgtaacatttctgaaaagatttttcagagcagatgagaagtatccattcctggtgcatccagtgatgccaatgaaagaaattcacgaatcaatcagatggaccaaggaccctagaaacacacaggatcacgtacgctcgttgtgcctattagcttggcacaacggtgaagaagaatacaataaatttttagctaaaatcagaagtgtgccaatcggaagagctttattgctcccagagtactctacattgtaccgccgatggctcgactcattttagtaaccctacctcagtcggattggattgggttatactgttgtaggggtaaatttttctttaattcggagaaaaaaaaaaaaaaaaaaagagctcccaatcactagtgaattcgcggccgcctgcaggtcgaccatatgggagagctcccaacgcgttggatgcatagcttgagtattctatagtgtcacctaaatagcttggcgtaatcatggtcatagctgtttcctgtgtgaaattgttatccgctcacaattccacacaacatacgagccggaagcataaagtgtaaagcctggggtgcctaatgagtgagctaactcacattaattgcgttgcgctcactgcccgctttccagtcgggaaacctgtcgtgccagctgcattaatgaatcggccaacgcgcggggagaggcggtttgcgtattgggcgctcttccgcttcctcgctcactgactcgctgcgctcggtcgttcggctgcggcgagcggtatcagctcactcaaaggcggtaatacggttatccacagaatcaggggataacgcaggaaagaacatgtgagcaaaaggccagcaaaaggccaggaaccgtaaaaaggccgcgttgctggcgtttttccataggctccgcccccctgacgagcatcacaaaaatcgacgctcaagtcagaggtggcgaaacccgacaggactataaagataccaggcgtttccccctggaagctccctcgtgcgctctcctgttccgaccctgccgcttaccggatacctgtccgcctttctcccttcgggaagcgtggcgctttctcatagctcacgctgtaggtatctcagttcggtgtaggtcgttcgctccaagctgggctgtgtgcacgaaccccccgttcagcccgaccgctgcgccttatccggtaactatcgtcttgagtccaacccggtaagacacgacttatcgccactggcagcagccactggtaacaggattagcagagcgaggtatgtaggcggtgctacagagttcttgaagtggtggcctaactacggctacactagaagaacagtatttggtatctgcgctctgctgaagccagttaccttcggaaaaagagttggtagctcttgatccggcaaacaaaccaccgctggtagcggtggtttttttgtttgcaagcagcagattacgcgcagaaaaaaaggatctcaagaagatcctttgatcttttctacggggtctgacgctcagtggaacgaaaactcacgttaagggattttggtcatgagattatcaaaaaggatcttcacctagatccttttaaattaaaaatgaagttttaaatcaatctaaagtatatatgagtaaacttggtctgacagttaccaatgcttaatcagtgaggcacctatctcagcgatctgtctatttcgttcatccatagttgcctgactccccgtcgtgtagataactacgatacgggagggcttaccatctggccccagtgctgcaatgataccgcgagacccacgctcaccggctccagatttatcagcaataaaccagccagccggaagggccgagcgcagaagtggtcctgcaactttatccgcctccatccagtctattaattgttgccgggaagctagagtaagtagttcgccagttaatagtttgcgcaacgttgttgccattgctacaggcatcgtggtgtcacgctcgtcgtttggtatggcttcattcagctccggttcccaacgatcaaggcgagttacatgatcccccatgttgtgcaaaaaagcggttagctccttcggtcctccgatcgttgtcagaagtaagttggccgcagtgttatcactcatggttatggcagcactgcataattctcttactgtcatgccatccgtaagatgcttttctgtgactggtgagtactcaaccaagtcattctgagaatagtgtatgcggcgaccgagttgctcttgcccggcgtcaatacgggataataccgcgccacatagcagaactttaaaagtgctcatcattggaaaacgttcttcggggcgaaaactctcaaggatcttaccgctgttgagatccagttcgatgtaacccactcgtgcacccaactgatcttcagcatcttttactttcaccagcgtttctgggtgagcaaaaacaggaaggcaaaatgccgcaaaaaagggaataagggcgacacggaaatgttgaatactcatactcttcctttttcaatattattgaagcatttatcagggttattgtctcatgagcggatacatatttgaatgtatttagaaaaataaacaaataggggttccgcgcacatttccccgaaaagtgccacctgatgcggtgtgaaataccgcacagatgcgtaaggagaaaataccgcatcaggaaattgtaagcgttaatattttgttaaaattcgcgttaaatttttgttaaatcagctcattttttaaccaataggccgaaatcggcaaaatcccttataaatcaaaagaatagaccgagatagggttgagtgttgttccagtttggaacaagagtccactattaaagaacgtggactccaacgtcaaagggcgaaaaaccgtctatcagggcgatggcccactacgtgaaccatcaccctaatcaagttttttggggtcgaggtgccgtaaagcactaaatcggaaccctaaagggagcccccgatttagagcttgacggggaaagccggcgaacgtggcgagaaaggaagggaagaaagcgaaaggagcgggcgctagggcgctggcaagtgtagcggtcacgctgcgcgtaaccaccacacccgccgcgcttaatgcgccgctacagggcgcgtccattcgccattcaggctgcgcaactgttgggaagggcgatcggtgcgggcctcttcgctattacgccagctggcgaaagggggatgtgctgcaaggcgattaagttgggtaacgccagggttttcccagtcacgacgttgtaaaacgacggccagtgaattgtaatacgactcactatagggcgaattgggcccgacgtcgcatgctcccggccgccatggcggccgcgggaattcgattgaggcatgctaatacgactcactatagg

SEQ ID NO: 8 - DNA, 10598 bp, artificial
  DNA encoding infectious nucleic acid
ttaaaacagctctggggttgttcccaccccagaggcccacgtggcggctagtactctggtattacggtacctttgtacgcctgttttgtatcccttcccccgtaactttagaagcttatcaaaagttcaatagcaggggtacaaaccagtacctctacgaacaagcacttctgtttccccggtgatatcacatagactgtacccacggtcaaaagtgattgatccgttatccgcttgagtacttcgagaagcctagtatcaccttggaatcttcgatgcgttgcgctcaacactctgccccgagtgtagcttaggctgatgagtctgggcactccccaccggcgacggtggcccaggctgcgttggcggcctacccatggctgatgccgtgggacgctagttgtgaacaaggtgtgaagagcctattgagctactcaagagtcctccggcccctgaatgcggctaatcctaaccacggagcaaccgctcacaacccagtgagtaggttgtcgtaatgcgtaagtctgtggcggaaccgactactttgggtgtccgtgtttccctttatattcatactggctgcttatggtgacaatttacaaattgttaccatatagctattggattggccacccagtattgtgcaatatatttgagtgtttctttcataagccttattaacatcggcgcgccgcacagctggttgaaggggaccaacgatacagctggttgaaggggaccaactggagccacacacttccttacattccatcacccacacacttccttacattccacggcgcgccacatttttaatcacaataaacagtgcaaatgggggctcaagtttcaacgcaaaagaccggtgcgcacgagaatcaaaacgtggcagccaatggatccaccattaattacactactatcaactattacaaagacagtgcgagtaattccgctactagacaagacctctcccaagatccatcaaaattcacagaaccggttaaggacttaatgttgaaaacagcaccagctctaaactcgcctaacgtggaagcatgtgggtacagtgaccgtgtgaggcaaatcactttaggcaactcgactattactacacaagaagcagccaatgctattgttgcttacggtgaatggcccacttacataaatgattcagaagctaatccggtagatgcacccactgagccagacgttagtagcaaccggttttacaccctagaatcggtgtcttggaagaccacttcaaggggatggtggtggaagttaccagattgtttgaaggacatgggaatgtttggtcagaatatgtactatcactacttggggcgctctggttacaccattcatgtccagtgcaacgcttcaaaatttcaccaaggggcgttaggagttttcctgataccagagtttgtcatggcttgcaacactgagagtaaaacgtcatacgtttcatacatcaatgcaaatcctggtgagagaggcggtgagtttacgaacacctacaatccgtcaaatacagacgccagtgagggcagaaagtttgcagcattggattatttgctgggttctggtgttctagcaggaaacgcctttgtgtacccgcaccagatcatcaacctacgtaccaacaacagtgcaacaattgtggtgccatacgtaaactcacttgtgattgattgtatggcaaaacacaataactggggcattgtcatattaccactggcacccttggcctttgccgcaacatcgtcaccacaggtgcctattacagtgaccattgcacccatgtgtacagaattcaatgggttgagaaacatcaccgtcccagtacatcaagggttgccgacaatgaacacacctggttccaatcaattccttacatctgatgacttccagtcgccctgtgccttacctaattttgatgttactccaccaatacacatacccggggaagtaaagaatatgatggaactagctgaaattgacacattgatcccaatgaacgcagtggacgggaaggtgaacacaatggagatgtatcaaataccattgaatgacaatttgagcaaggcacctatattctgtttatccctatcacctgcttctgataaacgactgagccacaccatgttgggtgaaatcctaaattattacacccattggacggggtccatcaggttcacctttctattttgtggcagtatgatggccactggtaaactgctcctcagctattccccaccgggagctaaaccaccaaccaatcgcaaggatgcaatgctaggcacacacatcatctgggacctagggttacaatccagttgttccatggttgcaccgtggatctccaacacagtgtacagacggtgtgcacgtgatgacttcactgagggcggatttataacttgcttctatcaaactagaattgtggtacctgcttcaacccctaccagtatgttcatgttaggctttgttagtgcgtgtccagacttcagtgtcagactgcttagggacactccccatattagtcaatcgaaactaataggacgtacacaaggcattgaagacctcattgacacagcgataaagaatgccttaagagtgtcccaaccaccctcgacccagtcaactgaagcaactagtggagtgaatagccaggaggtgccagctctaactgctgtggaaacaggagcatctggtcaagcaatccccagtgatgtggtggaaactaggcacgtggtaaattacaaaaccaggtctgaatcgtgtcttgagtcattctttgggagagctgcgtgtgtcacaatcctatccttgaccaactcctccaagagcggagaggagaaaaagcatttcaacatatggaatattacatacaccgacactgtccagttacgcagaaaattagaatttttcacgtattccaggtttgatcttgaaatgacttttgtattcacagagaactatcctagtacagccagtggagaagtgcgaaaccaggtgtaccagatcatgtatattccaccaggggcaccccgcccatcatcctgggatgactacacatggcaatcctcttcaaacccttccatcttctacatgtatggaaatgcacctccacggatgtcaattccttacgtagggattgccaatgcctattcacacttctacgatggctttgcacgggtgccacttgagggtgagaacaccgatgctggcgacacgttttacggtttagtgtccataaatgattttggagttttagcagttagagcagtaaaccgcagtaatccacatacaatacacacatctgtgagagtgtacatgaaaccaaaacacattcggtgttggtgccccagacctcctcgagctgtattatacaggggagagggagtggacatgatatccagtgcaattctacctctggccaaggtagactcaattaccacttttgggtttggtcatcagaacaaagcagtgtacgttgccggttacaagatttgcaactaccacctagcaaccccaagtgatcacttgaatgcaattagtatgttatgggacagggatttaatggtggtggaatctagagcccggggaactgataccatcgccagatgtagttgcaggtgtggagtttactattgtgaatctaggaggaagtactaccctgtcacttttactggcccaacgtttcgattcatggaagcaaacgactactatccagcaagataccagtctcacatgctgatagggtgcggatttgcagaacccggggactgcggtgggatactgaggtgcactcatggggtaattggtatcattactgcaggaggtgaaggggtagtagcctttgctgacattagagacctctgggtgtatgaagaggaggccatggaacagggaataacaagctacatcgaatctctcggcacagcctttggcgcagggttcacccacacaatcagtgagaaagtgactgaattgacaacgatggttaccagcactatcacagaaaaactactgaaaaacttggtgaaaatagtgtcggctctagtgattgttgtgagaaattatgaggacactaccacgatccttgcaacactagcactactcgggtgtgatatatctccttggcaatggttgaagaagaaggcatgtgacttactagagattccttatgtgatgcgccaaggtgatgggtggatgaagaaattcacagaggcgtgcaatgcagctaaaggcttagagtggattagcaacaaaatttccaagtttatagattggttgaagtgtaaaattatcccagacgctaaggacaaggtggaatttctcaccaagttgaaacagctagacatgttggaaaatcaaattgcaaccatccaccaatcttgccccagccaagaacaacaagagattcttttcaacaatgtgagatggttagcagtccagtcccgtcggtttgcaccattatacgctgtggaggcacgccgaattaacaaaatggagagcacaataaacaattatatacagttcaagagcaaacaccgtattgaaccagtatgtatgctcattcatgggtcaccagggacgggtaaatctatagctacttcattaataggtagagcaatagcagagaaggaaagcacatcagtctattcaatgccacctgacccatctcactttgatggctataaacaacaaggggtagtgattatggacgacctaaaccaaaaccccgatggtatggacatgaaactgttttgccaaatggtatcaacagtggagtttattcctccaatggcctcattagaggagaagggcattttgtttacatctgattatgtcctggcttctaccaactctcattcaattgtaccacccacagtggctcacagtgatgccttaaccagacgatttgcatttgatgtggaggtttacacgatgtctgaacattcagtcaaaggcaaactgaatatggccacggccactcaattgtgtaaggattgtccaacacctgcaaattttaaaaagtgttgccctctcgtttgtggaaaggccttgcaattaatggacaggtacaccagacaaaggttcactgtagatgagattaccacattaatcatgaatgagaaaaacagaagggccaatatcggcaattgcatggaagccttgtttcaaggaccactaaggtataaagatttgaagatcgatgtgaagacagttcccccccctgagtgcatcagtgatttgttacaagcagtggattctcaagaggttagggattactgtgagaagaaaggctggatcgttaacgttactagccagattcaactagaaaggaacatcaatagggccatgactatactccaagctgttaccacattcgcagcagtcgcaggagtagtgtatgtaatgtacaaactcttcgccggtcaacagggtgcatacactggcttgccaaacaaaaaacccaatgtccctactatcagagtcgctaaagtccaggggccaggatttgactacgcagtggcaatggcaaaaagaaacatagttactgcaaccaccaccaagggtgaatttaccatgctaggggtgcatgataatgtagcaatattgccaacccatgccgctccaggagaaaccattattattgatgggaaagaagtagagatcctagacgccagagccttagaagatcaagcgggaaccaatcttgagatcaccattattactctaaaaagaaatgagaagtttagagacatcagatcacatattcccacccaaattactgaaactaacgatggagtgttgatcgtgaacactagcaagtaccccaatatgtatgtccccgttggtgctgtgaccgaacagggatatcttaatctcagtggacgtcaaactgctcgcactttaatgtacaactttccaacaagggcaggccagtgcggaggaatcatcacttgtactggcaaagtcattgggatgcatgttggcgggaacggttcacatgggtttgctgcagccctcaagcgatcatacttcactcaaaatcagggcgaaatccagtggatgaggtcatcaaaagaagtggggtaccccattataaatgccccatccaagacaaagttagaacccagtgctttccactatgtttttgaaggtgttaaggaaccagctgtactcactaagaatgaccccagactaaaaacagattttgaagaagccatcttttctaaatatgtggggaacaaaattactgaagtggacgagtacatgaaagaagcagtggatcactatgcaggacagttaatgtcactggatatcaacacagaacagatgtgcctggaggatgccatgtacggtaccgatggtcttgaggccctggatcttagcactagtgctggatatccttatgttgcaatggggaaaaagaaaagagacattctagataaacagaccagagatactaaggagatgcagagacttttagatacctatggaatcaatctaccattagtcacgtacgtgaaagatgaactcaggtcaaagactaaagtggaacaaggaaagtcaagattgattgaagcttccagccttaatgattcagttgcaatgagaatggcctttggcaatctttacgcagctttccacaagaatccaggtgtggtgacaggatcagcagttggttgtgacccagatttgttttggagtaagataccagtgctaatggaagaaaaactcttcgcttttgactacacagggtatgatgcctcactcagccctgcttggtttgaagctcttaaaatggtgttagaaaaaattggatttggcagtagagtagactatatagactacctgaaccactctcaccacctttacaaaaacaagacttattgtgtcaaaggcggcatgccatccggctgctctggcacctcaattttcaactcaatgattaacaacctgatcattaggacgcttttactgagaacctacaagggcatagacttggaccatttaaaaatgattgcctatggtgatgacgtgatagcttcctacccccatgaggttgacgctagtctcctagcccaatcaggaaaagactatggactaaccatgactccagcagataaatcagcaacctttgaaacagtcacatgggagaatgtaacatttctgaaaagatttttcagagcagatgagaagtatccattcctggtgcatccagtgatgccaatgaaagaaattcacgaatcaatcagatggaccaaggaccctagaaacacacaggatcacgtacgctcgttgtgcctattagcttggcacaacggtgaagaagaatacaataaatttttagctaaaatcagaagtgtgccaatcggaagagctttattgctcccagagtactctacattgtaccgccgatggctcgactcattttagtaaccctacctcagtcggattggattgggttatactgttgtaggggtaaatttttctttaattcggagaaaaaaaaaaaaaaaaaaagagctcccaatcactagtgaattcgcggccgcctgcaggtcgaccatatgggagagctcccaacgcgttggatgcatagcttgagtattctatagtgtcacctaaatagcttggcgtaatcatggtcatagctgtttcctgtgtgaaattgttatccgctcacaattccacacaacatacgagccggaagcataaagtgtaaagcctggggtgcctaatgagtgagctaactcacattaattgcgttgcgctcactgcccgctttccagtcgggaaacctgtcgtgccagctgcattaatgaatcggccaacgcgcggggagaggcggtttgcgtattgggcgctcttccgcttcctcgctcactgactcgctgcgctcggtcgttcggctgcggcgagcggtatcagctcactcaaaggcggtaatacggttatccacagaatcaggggataacgcaggaaagaacatgtgagcaaaaggccagcaaaaggccaggaaccgtaaaaaggccgcgttgctggcgtttttccataggctccgcccccctgacgagcatcacaaaaatcgacgctcaagtcagaggtggcgaaacccgacaggactataaagataccaggcgtttccccctggaagctccctcgtgcgctctcctgttccgaccctgccgcttaccggatacctgtccgcctttctcccttcgggaagcgtggcgctttctcatagctcacgctgtaggtatctcagttcggtgtaggtcgttcgctccaagctgggctgtgtgcacgaaccccccgttcagcccgaccgctgcgccttatccggtaactatcgtcttgagtccaacccggtaagacacgacttatcgccactggcagcagccactggtaacaggattagcagagcgaggtatgtaggcggtgctacagagttcttgaagtggtggcctaactacggctacactagaagaacagtatttggtatctgcgctctgctgaagccagttaccttcggaaaaagagttggtagctcttgatccggcaaacaaaccaccgctggtagcggtggtttttttgtttgcaagcagcagattacgcgcagaaaaaaaggatctcaagaagatcctttgatcttttctacggggtctgacgctcagtggaacgaaaactcacgttaagggattttggtcatgagattatcaaaaaggatcttcacctagatccttttaaattaaaaatgaagttttaaatcaatctaaagtatatatgagtaaacttggtctgacagttaccaatgcttaatcagtgaggcacctatctcagcgatctgtctatttcgttcatccatagttgcctgactccccgtcgtgtagataactacgatacgggagggcttaccatctggccccagtgctgcaatgataccgcgagacccacgctcaccggctccagatttatcagcaataaaccagccagccggaagggccgagcgcagaagtggtcctgcaactttatccgcctccatccagtctattaattgttgccgggaagctagagtaagtagttcgccagttaatagtttgcgcaacgttgttgccattgctacaggcatcgtggtgtcacgctcgtcgtttggtatggcttcattcagctccggttcccaacgatcaaggcgagttacatgatcccccatgttgtgcaaaaaagcggttagctccttcggtcctccgatcgttgtcagaagtaagttggccgcagtgttatcactcatggttatggcagcactgcataattctcttactgtcatgccatccgtaagatgcttttctgtgactggtgagtactcaaccaagtcattctgagaatagtgtatgcggcgaccgagttgctcttgcccggcgtcaatacgggataataccgcgccacatagcagaactttaaaagtgctcatcattggaaaacgttcttcggggcgaaaactctcaaggatcttaccgctgttgagatccagttcgatgtaacccactcgtgcacccaactgatcttcagcatcttttactttcaccagcgtttctgggtgagcaaaaacaggaaggcaaaatgccgcaaaaaagggaataagggcgacacggaaatgttgaatactcatactcttcctttttcaatattattgaagcatttatcagggttattgtctcatgagcggatacatatttgaatgtatttagaaaaataaacaaataggggttccgcgcacatttccccgaaaagtgccacctgatgcggtgtgaaataccgcacagatgcgtaaggagaaaataccgcatcaggaaattgtaagcgttaatattttgttaaaattcgcgttaaatttttgttaaatcagctcattttttaaccaataggccgaaatcggcaaaatcccttataaatcaaaagaatagaccgagatagggttgagtgttgttccagtttggaacaagagtccactattaaagaacgtggactccaacgtcaaagggcgaaaaaccgtctatcagggcgatggcccactacgtgaaccatcaccctaatcaagttttttggggtcgaggtgccgtaaagcactaaatcggaaccctaaagggagcccccgatttagagcttgacggggaaagccggcgaacgtggcgagaaaggaagggaagaaagcgaaaggagcgggcgctagggcgctggcaagtgtagcggtcacgctgcgcgtaaccaccacacccgccgcgcttaatgcgccgctacagggcgcgtccattcgccattcaggctgcgcaactgttgggaagggcgatcggtgcgggcctcttcgctattacgccagctggcgaaagggggatgtgctgcaaggcgattaagttgggtaacgccagggttttcccagtcacgacgttgtaaaacgacggccagtgaattgtaatacgactcactatagggcgaattgggcccgacgtcgcatgctcccggccgccatggcggccgcgggaattcgattgaggcatgctaatacgactcactatagg

SEQ ID NO: 9 - DNA, 10561 bp, artificial
  DNA encoding infectious nucleic acid
ttaaaacagctctggggttgttcccaccccagaggcccacgtggcggctagtactctggtattacggtacctttgtacgcctgttttgtatcccttcccccgtaactttagaagcttatcaaaagttcaatagcaggggtacaaaccagtacctctacgaacaagcacttctgtttccccggtgatatcacatagactgtacccacggtcaaaagtgattgatccgttatccgcttgagtacttcgagaagcctagtatcaccttggaatcttcgatgcgttgcgctcaacactctgccccgagtgtagcttaggctgatgagtctgggcactccccaccggcgacggtggcccaggctgcgttggcggcctacccatggctgatgccgtgggacgctagttgtgaacaaggtgtgaagagcctattgagctactcaagagtcctccggcccctgaatgcggctaatcctaaccacggagcaaccgctcacaacccagtgagtaggttgtcgtaatgcgtaagtctgtggcggaaccgactactttgggtgtccgtgtttccctttatattcatactggctgcttatggtgacaatttacaaattgttaccatatagctattggattggccacccagtattgtgcaatatatttgagtgtttctttcataagccttattaacatcacatttttaatcacaataaacagtgcaaatgggggctcaagtttcaacgcaaaagaccggtgcgcacgagaatcaaaacgtggcagccaatggatccaccattaattacactactatcaactattacaaagacagtgcgagtaattccgctactagacaagacctctcccaagatccatcaaaattcacagaaccggttaaggacttaatgttgaaaacagcaccagctctaaactcgcctaacgtggaagcatgtgggtacagtgaccgtgtgaggcaaatcactttaggcaactcgactattactacacaagaagcagccaatgctattgttgcttacggtgaatggcccacttacataaatgattcagaagctaatccggtagatgcacccactgagccagacgttagtagcaaccggttttacaccctagaatcggtgtcttggaagaccacttcaaggggatggtggtggaagttaccagattgtttgaaggacatgggaatgtttggtcagaatatgtactatcactacttggggcgctctggttacaccattcatgtccagtgcaacgcttcaaaatttcaccaaggggcgttaggagttttcctgataccagagtttgtcatggcttgcaacactgagagtaaaacgtcatacgtttcatacatcaatgcaaatcctggtgagagaggcggtgagtttacgaacacctacaatccgtcaaatacagacgccagtgagggcagaaagtttgcagcattggattatttgctgggttctggtgttctagcaggaaacgcctttgtgtacccgcaccagatcatcaacctacgtaccaacaacagtgcaacaattgtggtgccatacgtaaactcacttgtgattgattgtatggcaaaacacaataactggggcattgtcatattaccactggcacccttggcctttgccgcaacatcgtcaccacaggtgcctattacagtgaccattgcacccatgtgtacagaattcaatgggttgagaaacatcaccgtcccagtacatcaagggttgccgacaatgaacacacctggttccaatcaattccttacatctgatgacttccagtcgccctgtgccttacctaattttgatgttactccaccaatacacatacccggggaagtaaagaatatgatggaactagctgaaattgacacattgatcccaatgaacgcagtggacgggaaggtgaacacaatggagatgtatcaaataccattgaatgacaatttgagcaaggcacctatattctgtttatccctatcacctgcttctgataaacgactgagccacaccatgttgggtgaaatcctaaattattacacccattggacggggtccatcaggttcacctttctattttgtggcagtatgatggccactggtaaactgctcctcagctattccccaccgggagctaaaccaccaaccaatcgcaaggatgcaatgctaggcacacacatcatctgggacctagggttacaatccagttgttccatggttgcaccgtggatctccaacacagtgtacagacggtgtgcacgtgatgacttcactgagggcggatttataacttgcttctatcaaactagaattgtggtacctgcttcaacccctaccagtatgttcatgttaggctttgttagtgcgtgtccagacttcagtgtcagactgcttagggacactccccatattagtcaatcgaaactaataggacgtacacaaggcattgaagacctcattgacacagcgataaagaatgccttaagagtgtcccaaccaccctcgacccagtcaactgaagcaactagtggagtgaatagccaggaggtgccagctctaactgctgtggaaacaggagcatctggtcaagcaatccccagtgatgtggtggaaactaggcacgtggtaaattacaaaaccaggtctgaatcgtgtcttgagtcattctttgggagagctgcgtgtgtcacaatcctatccttgaccaactcctccaagagcggagaggagaaaaagcatttcaacatatggaatattacatacaccgacactgtccagttacgcagaaaattagaatttttcacgtattccaggtttgatcttgaaatgacttttgtattcacagagaactatcctagtacagccagtggagaagtgcgaaaccaggtgtaccagatcatgtatattccaccaggggcaccccgcccatcatcctgggatgactacacatggcaatcctcttcaaacccttccatcttctacatgtatggaaatgcacctccacggatgtcaattccttacgtagggattgccaatgcctattcacacttctacgatggctttgcacgggtgccacttgagggtgagaacaccgatgctggcgacacgttttacggtttagtgtccataaatgattttggagttttagcagttagagcagtaaaccgcagtaatccacatacaatacacacatctgtgagagtgtacatgaaaccaaaacacattcggtgttggtgccccagacctcctcgagctgtattatacaggggagagggagtggacatgatatccagtgcaattctacctctggccaaggtagactcaattaccacttttgggtttggtcatcagaacaaagcagtgtacgttgccggttacaagatttgcaactaccacctagcaaccccaagtgatcacttgaatgcaattagtatgttatgggacagggatttaatggtggtggaatctagagcccggggaactgataccatcgccagatgtagttgcaggtgtggagtttactattgtgaatctaggaggaagtactaccctgtcacttttactggcccaacgtttcgattcatggaagcaaacgactactatccagcaagataccagtctcacatgctgatagggtgcggatttgcagaacccggggactgcggtgggatactgaggtgcactcatggggtaattggtatcattactgcaggaggtgaaggggtagtagcctttgctgacattagagacctctgggtgtatgaagaggaggccatggaacagggaataacaagctacatcgaatctctcggcacagcctttggcgcagggttcacccacacaatcagtgagaaagtgactgaattgacaacgatggttaccagcactatcacagaaaaactactgaaaaacttggtgaaaatagtgtcggctctagtgattgttgtgagaaattatgaggacactaccacgatccttgcaacactagcactactcgggtgtgatatatctccttggcaatggttgaagaagaaggcatgtgacttactagagattccttatgtgatgcgccaaggtgatgggtggatgaagaaattcacagaggcgtgcaatgcagctaaaggcttagagtggattagcaacaaaatttccaagtttatagattggttgaagtgtaaaattatcccagacgctaaggacaaggtggaatttctcaccaagttgaaacagctagacatgttggaaaatcaaattgcaaccatccaccaatcttgccccagccaagaacaacaagagattcttttcaacaatgtgagatggttagcagtccagtcccgtcggtttgcaccattatacgctgtggaggcacgccgaattaacaaaatggagagcacaataaacaattatatacagttcaagagcaaacaccgtattgaaccagtatgtatgctcattcatgggtcaccagggacgggtaaatctatagctacttcattaataggtagagcaatagcagagaaggaaagcacatcagtctattcaatgccacctgacccatctcactttgatggctataaacaacaaggggtagtgattatggacgacctaaaccaaaaccccgatggtatggacatgaaactgttttgccaaatggtatcaacagtggagtttattcctccaatggcctcattagaggagaagggcattttgtttacatctgattatgtcctggcttctaccaactctcattcaattgtaccacccacagtggctcacagtgatgccttaaccagacgatttgcatttgatgtggaggtttacacgatgtctgaacattcagtcaaaggcaaactgaatatggccacggccactcaattgtgtaaggattgtccaacacctgcaaattttaaaaagtgttgccctctcgtttgtggaaaggccttgcaattaatggacaggtacaccagacaaaggttcactgtagatgagattaccacattaatcatgaatgagaaaaacagaagggccaatatcggcaattgcatggaagccttgtttcaaggaccactaaggtataaagatttgaagatcgatgtgaagacagttcccccccctgagtgcatcagtgatttgttacaagcagtggattctcaagaggttagggattactgtgagaagaaaggctggatcgttaacgttactagccagattcaactagaaaggaacatcaatagggccatgactatactccaagctgttaccacattcgcagcagtcgcaggagtagtgtatgtaatgtacaaactcttcgccggtcaacagggtgcatacactggcttgccaaacaaaaaacccaatgtccctactatcagagtcgctaaagtccaggggccaggatttgactacgcagtggcaatggcaaaaagaaacatagttactgcaaccaccaccaagggtgaatttaccatgctaggggtgcatgataatgtagcaatattgccaacccatgccgctccaggagaaaccattattattgatgggaaagaagtagagatcctagacgccagagccttagaagatcaagcgggaaccaatcttgagatcaccattattactctaaaaagaaatgagaagtttagagacatcagatcacatattcccacccaaattactgaaactaacgatggagtgttgatcgtgaacactagcaagtaccccaatatgtatgtccccgttggtgctgtgaccgaacagggatatcttaatctcagtggacgtcaaactgctcgcactttaatgtacaactttccaacaagggcaggccagtgcggaggaatcatcacttgtactggcaaagtcattgggatgcatgttggcgggaacggttcacatgggtttgctgcagccctcaagcgatcatacttcactcaaaatcagggcgaaatccagtggatgaggtcatcaaaagaagtggggtaccccattataaatgccccatccaagacaaagttagaacccagtgctttccactatgtttttgaaggtgttaaggaaccagctgtactcactaagaatgaccccagactaaaaacagattttgaagaagccatcttttctaaatatgtggggaacaaaattactgaagtggacgagtacatgaaagaagcagtggatcactatgcaggacagttaatgtcactggatatcaacacagaacagatgtgcctggaggatgccatgtacggtaccgatggtcttgaggccctggatcttagcactagtgctggatatccttatgttgcaatggggaaaaagaaaagagacattctagataaacagaccagagatactaaggagatgcagagacttttagatacctatggaatcaatctaccattagtcacgtacgtgaaagatgaactcaggtcaaagactaaagtggaacaaggaaagtcaagattgattgaagcttccagccttaatgattcagttgcaatgagaatggcctttggcaatctttacgcagctttccacaagaatccaggtgtggtgacaggatcagcagttggttgtgacccagatttgttttggagtaagataccagtgctaatggaagaaaaactcttcgcttttgactacacagggtatgatgcctcactcagccctgcttggtttgaagctcttaaaatggtgttagaaaaaattggatttggcagtagagtagactatatagactacctgaaccactctcaccacctttacaaaaacaagacttattgtgtcaaaggcggcatgccatccggctgctctggcacctcaattttcaactcaatgattaacaacctgatcattaggacgcttttactgagaacctacaagggcatagacttggaccatttaaaaatgattgcctatggtgatgacgtgatagcttcctacccccatgaggttgacgctagtctcctagcccaatcaggaaaagactatggactaaccatgactccagcagataaatcagcaacctttgaaacagtcacatgggagaatgtaacatttctgaaaagatttttcagagcagatgagaagtatccattcctggtgcatccagtgatgccaatgaaagaaattcacgaatcaatcagatggaccaaggaccctagaaacacacaggatcacgtacgctcgttgtgcctattagcttggcacaacggtgaagaagaatacaataaatttttagctaaaatcagaagtgtgccaatcggaagagctttattgctcccagagtactctacattgtaccgccgatggctcgactcattttagtaaggcgcgccgcacagctggttgaaggggaccaactggagccacacacttccttacattccacggcgcgccgactcattttagtaaccctacctcagtcggattggattgggttatactgttgtaggggtaaatttttctttaattcggagaaaaaaaaaaaaaaaaaaagagctcccaatcactagtgaattcgcggccgcctgcaggtcgaccatatgggagagctcccaacgcgttggatgcatagcttgagtattctatagtgtcacctaaatagcttggcgtaatcatggtcatagctgtttcctgtgtgaaattgttatccgctcacaattccacacaacatacgagccggaagcataaagtgtaaagcctggggtgcctaatgagtgagctaactcacattaattgcgttgcgctcactgcccgctttccagtcgggaaacctgtcgtgccagctgcattaatgaatcggccaacgcgcggggagaggcggtttgcgtattgggcgctcttccgcttcctcgctcactgactcgctgcgctcggtcgttcggctgcggcgagcggtatcagctcactcaaaggcggtaatacggttatccacagaatcaggggataacgcaggaaagaacatgtgagcaaaaggccagcaaaaggccaggaaccgtaaaaaggccgcgttgctggcgtttttccataggctccgcccccctgacgagcatcacaaaaatcgacgctcaagtcagaggtggcgaaacccgacaggactataaagataccaggcgtttccccctggaagctccctcgtgcgctctcctgttccgaccctgccgcttaccggatacctgtccgcctttctcccttcgggaagcgtggcgctttctcatagctcacgctgtaggtatctcagttcggtgtaggtcgttcgctccaagctgggctgtgtgcacgaaccccccgttcagcccgaccgctgcgccttatccggtaactatcgtcttgagtccaacccggtaagacacgacttatcgccactggcagcagccactggtaacaggattagcagagcgaggtatgtaggcggtgctacagagttcttgaagtggtggcctaactacggctacactagaagaacagtatttggtatctgcgctctgctgaagccagttaccttcggaaaaagagttggtagctcttgatccggcaaacaaaccaccgctggtagcggtggtttttttgtttgcaagcagcagattacgcgcagaaaaaaaggatctcaagaagatcctttgatcttttctacggggtctgacgctcagtggaacgaaaactcacgttaagggattttggtcatgagattatcaaaaaggatcttcacctagatccttttaaattaaaaatgaagttttaaatcaatctaaagtatatatgagtaaacttggtctgacagttaccaatgcttaatcagtgaggcacctatctcagcgatctgtctatttcgttcatccatagttgcctgactccccgtcgtgtagataactacgatacgggagggcttaccatctggccccagtgctgcaatgataccgcgagacccacgctcaccggctccagatttatcagcaataaaccagccagccggaagggccgagcgcagaagtggtcctgcaactttatccgcctccatccagtctattaattgttgccgggaagctagagtaagtagttcgccagttaatagtttgcgcaacgttgttgccattgctacaggcatcgtggtgtcacgctcgtcgtttggtatggcttcattcagctccggttcccaacgatcaaggcgagttacatgatcccccatgttgtgcaaaaaagcggttagctccttcggtcctccgatcgttgtcagaagtaagttggccgcagtgttatcactcatggttatggcagcactgcataattctcttactgtcatgccatccgtaagatgcttttctgtgactggtgagtactcaaccaagtcattctgagaatagtgtatgcggcgaccgagttgctcttgcccggcgtcaatacgggataataccgcgccacatagcagaactttaaaagtgctcatcattggaaaacgttcttcggggcgaaaactctcaaggatcttaccgctgttgagatccagttcgatgtaacccactcgtgcacccaactgatcttcagcatcttttactttcaccagcgtttctgggtgagcaaaaacaggaaggcaaaatgccgcaaaaaagggaataagggcgacacggaaatgttgaatactcatactcttcctttttcaatattattgaagcatttatcagggttattgtctcatgagcggatacatatttgaatgtatttagaaaaataaacaaataggggttccgcgcacatttccccgaaaagtgccacctgatgcggtgtgaaataccgcacagatgcgtaaggagaaaataccgcatcaggaaattgtaagcgttaatattttgttaaaattcgcgttaaatttttgttaaatcagctcattttttaaccaataggccgaaatcggcaaaatcccttataaatcaaaagaatagaccgagatagggttgagtgttgttccagtttggaacaagagtccactattaaagaacgtggactccaacgtcaaagggcgaaaaaccgtctatcagggcgatggcccactacgtgaaccatcaccctaatcaagttttttggggtcgaggtgccgtaaagcactaaatcggaaccctaaagggagcccccgatttagagcttgacggggaaagccggcgaacgtggcgagaaaggaagggaagaaagcgaaaggagcgggcgctagggcgctggcaagtgtagcggtcacgctgcgcgtaaccaccacacccgccgcgcttaatgcgccgctacagggcgcgtccattcgccattcaggctgcgcaactgttgggaagggcgatcggtgcgggcctcttcgctattacgccagctggcgaaagggggatgtgctgcaaggcgattaagttgggtaacgccagggttttcccagtcacgacgttgtaaaacgacggccagtgaattgtaatacgactcactatagggcgaattgggcccgacgtcgcatgctcccggccgccatggcggccgcgggaattcgattgaggcatgctaatacgactcactatagg

SEQ ID NO: 10 - DNA, 10613 bp, artificial
  DNA encoding infectious nucleic acid
ttaaaacagctctggggttgttcccaccccagaggcccacgtggcggctagtactctggtattacggtacctttgtacgcctgttttgtatcccttcccccgtaactttagaagcttatcaaaagttcaatagcaggggtacaaaccagtacctctacgaacaagcacttctgtttccccggtgatatcacatagactgtacccacggtcaaaagtgattgatccgttatccgcttgagtacttcgagaagcctagtatcaccttggaatcttcgatgcgttgcgctcaacactctgccccgagtgtagcttaggctgatgagtctgggcactccccaccggcgacggtggcccaggctgcgttggcggcctacccatggctgatgccgtgggacgctagttgtgaacaaggtgtgaagagcctattgagctactcaagagtcctccggcccctgaatgcggctaatcctaaccacggagcaaccgctcacaacccagtgagtaggttgtcgtaatgcgtaagtctgtggcggaaccgactactttgggtgtccgtgtttccctttatattcatactggctgcttatggtgacaatttacaaattgttaccatatagctattggattggccacccagtattgtgcaatatatttgagtgtttctttcataagccttattaacatcacatttttaatcacaataaacagtgcaaatgggggctcaagtttcaacgcaaaagaccggtgcgcacgagaatcaaaacgtggcagccaatggatccaccattaattacactactatcaactattacaaagacagtgcgagtaattccgctactagacaagacctctcccaagatccatcaaaattcacagaaccggttaaggacttaatgttgaaaacagcaccagctctaaactcgcctaacgtggaagcatgtgggtacagtgaccgtgtgaggcaaatcactttaggcaactcgactattactacacaagaagcagccaatgctattgttgcttacggtgaatggcccacttacataaatgattcagaagctaatccggtagatgcacccactgagccagacgttagtagcaaccggttttacaccctagaatcggtgtcttggaagaccacttcaaggggatggtggtggaagttaccagattgtttgaaggacatgggaatgtttggtcagaatatgtactatcactacttggggcgctctggttacaccattcatgtccagtgcaacgcttcaaaatttcaccaaggggcgttaggagttttcctgataccagagtttgtcatggcttgcaacactgagagtaaaacgtcatacgtttcatacatcaatgcaaatcctggtgagagaggcggtgagtttacgaacacctacaatccgtcaaatacagacgccagtgagggcagaaagtttgcagcattggattatttgctgggttctggtgttctagcaggaaacgcctttgtgtacccgcaccagatcatcaacctacgtaccaacaacagtgcaacaattgtggtgccatacgtaaactcacttgtgattgattgtatggcaaaacacaataactggggcattgtcatattaccactggcacccttggcctttgccgcaacatcgtcaccacaggtgcctattacagtgaccattgcacccatgtgtacagaattcaatgggttgagaaacatcaccgtcccagtacatcaagggttgccgacaatgaacacacctggttccaatcaattccttacatctgatgacttccagtcgccctgtgccttacctaattttgatgttactccaccaatacacatacccggggaagtaaagaatatgatggaactagctgaaattgacacattgatcccaatgaacgcagtggacgggaaggtgaacacaatggagatgtatcaaataccattgaatgacaatttgagcaaggcacctatattctgtttatccctatcacctgcttctgataaacgactgagccacaccatgttgggtgaaatcctaaattattacacccattggacggggtccatcaggttcacctttctattttgtggcagtatgatggccactggtaaactgctcctcagctattccccaccgggagctaaaccaccaaccaatcgcaaggatgcaatgctaggcacacacatcatctgggacctagggttacaatccagttgttccatggttgcaccgtggatctccaacacagtgtacagacggtgtgcacgtgatgacttcactgagggcggatttataacttgcttctatcaaactagaattgtggtacctgcttcaacccctaccagtatgttcatgttaggctttgttagtgcgtgtccagacttcagtgtcagactgcttagggacactccccatattagtcaatcgaaactaataggacgtacacaaggcattgaagacctcattgacacagcgataaagaatgccttaagagtgtcccaaccaccctcgacccagtcaactgaagcaactagtggagtgaatagccaggaggtgccagctctaactgctgtggaaacaggagcatctggtcaagcaatccccagtgatgtggtggaaactaggcacgtggtaaattacaaaaccaggtctgaatcgtgtcttgagtcattctttgggagagctgcgtgtgtcacaatcctatccttgaccaactcctccaagagcggagaggagaaaaagcatttcaacatatggaatattacatacaccgacactgtccagttacgcagaaaattagaatttttcacgtattccaggtttgatcttgaaatgacttttgtattcacagagaactatcctagtacagccagtggagaagtgcgaaaccaggtgtaccagatcatgtatattccaccaggggcaccccgcccatcatcctgggatgactacacatggcaatcctcttcaaacccttccatcttctacatgtatggaaatgcacctccacggatgtcaattccttacgtagggattgccaatgcctattcacacttctacgatggctttgcacgggtgccacttgagggtgagaacaccgatgctggcgacacgttttacggtttagtgtccataaatgattttggagttttagcagttagagcagtaaaccgcagtaatccacatacaatacacacatctgtgagagtgtacatgaaaccaaaacacattcggtgttggtgccccagacctcctcgagctgtattatacaggggagagggagtggacatgatatccagtgcaattctacctctggccaaggtagactcaattaccacttttgggtttggtcatcagaacaaagcagtgtacgttgccggttacaagatttgcaactaccacctagcaaccccaagtgatcacttgaatgcaattagtatgttatgggacagggatttaatggtggtggaatctagagcccggggaactgataccatcgccagatgtagttgcaggtgtggagtttactattgtgaatctaggaggaagtactaccctgtcacttttactggcccaacgtttcgattcatggaagcaaacgactactatccagcaagataccagtctcacatgctgatagggtgcggatttgcagaacccggggactgcggtgggatactgaggtgcactcatggggtaattggtatcattactgcaggaggtgaaggggtagtagcctttgctgacattagagacctctgggtgtatgaagaggaggccatggaacagggaataacaagctacatcgaatctctcggcacagcctttggcgcagggttcacccacacaatcagtgagaaagtgactgaattgacaacgatggttaccagcactatcacagaaaaactactgaaaaacttggtgaaaatagtgtcggctctagtgattgttgtgagaaattatgaggacactaccacgatccttgcaacactagcactactcgggtgtgatatatctccttggcaatggttgaagaagaaggcatgtgacttactagagattccttatgtgatgcgccaaggtgatgggtggatgaagaaattcacagaggcgtgcaatgcagctaaaggcttagagtggattagcaacaaaatttccaagtttatagattggttgaagtgtaaaattatcccagacgctaaggacaaggtggaatttctcaccaagttgaaacagctagacatgttggaaaatcaaattgcaaccatccaccaatcttgccccagccaagaacaacaagagattcttttcaacaatgtgagatggttagcagtccagtcccgtcggtttgcaccattatacgctgtggaggcacgccgaattaacaaaatggagagcacaataaacaattatatacagttcaagagcaaacaccgtattgaaccagtatgtatgctcattcatgggtcaccagggacgggtaaatctatagctacttcattaataggtagagcaatagcagagaaggaaagcacatcagtctattcaatgccacctgacccatctcactttgatggctataaacaacaaggggtagtgattatggacgacctaaaccaaaaccccgatggtatggacatgaaactgttttgccaaatggtatcaacagtggagtttattcctccaatggcctcattagaggagaagggcattttgtttacatctgattatgtcctggcttctaccaactctcattcaattgtaccacccacagtggctcacagtgatgccttaaccagacgatttgcatttgatgtggaggtttacacgatgtctgaacattcagtcaaaggcaaactgaatatggccacggccactcaattgtgtaaggattgtccaacacctgcaaattttaaaaagtgttgccctctcgtttgtggaaaggccttgcaattaatggacaggtacaccagacaaaggttcactgtagatgagattaccacattaatcatgaatgagaaaaacagaagggccaatatcggcaattgcatggaagccttgtttcaaggaccactaaggtataaagatttgaagatcgatgtgaagacagttcccccccctgagtgcatcagtgatttgttacaagcagtggattctcaagaggttagggattactgtgagaagaaaggctggatcgttaacgttactagccagattcaactagaaaggaacatcaatagggccatgactatactccaagctgttaccacattcgcagcagtcgcaggagtagtgtatgtaatgtacaaactcttcgccggtcaacagggtgcatacactggcttgccaaacaaaaaacccaatgtccctactatcagagtcgctaaagtccaggggccaggatttgactacgcagtggcaatggcaaaaagaaacatagttactgcaaccaccaccaagggtgaatttaccatgctaggggtgcatgataatgtagcaatattgccaacccatgccgctccaggagaaaccattattattgatgggaaagaagtagagatcctagacgccagagccttagaagatcaagcgggaaccaatcttgagatcaccattattactctaaaaagaaatgagaagtttagagacatcagatcacatattcccacccaaattactgaaactaacgatggagtgttgatcgtgaacactagcaagtaccccaatatgtatgtccccgttggtgctgtgaccgaacagggatatcttaatctcagtggacgtcaaactgctcgcactttaatgtacaactttccaacaagggcaggccagtgcggaggaatcatcacttgtactggcaaagtcattgggatgcatgttggcgggaacggttcacatgggtttgctgcagccctcaagcgatcatacttcactcaaaatcagggcgaaatccagtggatgaggtcatcaaaagaagtggggtaccccattataaatgccccatccaagacaaagttagaacccagtgctttccactatgtttttgaaggtgttaaggaaccagctgtactcactaagaatgaccccagactaaaaacagattttgaagaagccatcttttctaaatatgtggggaacaaaattactgaagtggacgagtacatgaaagaagcagtggatcactatgcaggacagttaatgtcactggatatcaacacagaacagatgtgcctggaggatgccatgtacggtaccgatggtcttgaggccctggatcttagcactagtgctggatatccttatgttgcaatggggaaaaagaaaagagacattctagataaacagaccagagatactaaggagatgcagagacttttagatacctatggaatcaatctaccattagtcacgtacgtgaaagatgaactcaggtcaaagactaaagtggaacaaggaaagtcaagattgattgaagcttccagccttaatgattcagttgcaatgagaatggcctttggcaatctttacgcagctttccacaagaatccaggtgtggtgacaggatcagcagttggttgtgacccagatttgttttggagtaagataccagtgctaatggaagaaaaactcttcgcttttgactacacagggtatgatgcctcactcagccctgcttggtttgaagctcttaaaatggtgttagaaaaaattggatttggcagtagagtagactatatagactacctgaaccactctcaccacctttacaaaaacaagacttattgtgtcaaaggcggcatgccatccggctgctctggcacctcaattttcaactcaatgattaacaacctgatcattaggacgcttttactgagaacctacaagggcatagacttggaccatttaaaaatgattgcctatggtgatgacgtgatagcttcctacccccatgaggttgacgctagtctcctagcccaatcaggaaaagactatggactaaccatgactccagcagataaatcagcaacctttgaaacagtcacatgggagaatgtaacatttctgaaaagatttttcagagcagatgagaagtatccattcctggtgcatccagtgatgccaatgaaagaaattcacgaatcaatcagatggaccaaggaccctagaaacacacaggatcacgtacgctcgttgtgcctattagcttggcacaacggtgaagaagaatacaataaatttttagctaaaatcagaagtgtgccaatcggaagagctttattgctcccagagtactctacattgtaccgccgatggctcgactcattttagtaaggcgcgccgcacagctggttgaaggggaccaacgatacagctggttgaaggggaccaactggagccacacacttccttacattccatcacccacacacttccttacattccacggcgcgccgactcattttagtaaccctacctcagtcggattggattgggttatactgttgtaggggtaaatttttctttaattcggagaaaaaaaaaaaaaaaaaaagagctcccaatcactagtgaattcgcggccgcctgcaggtcgaccatatgggagagctcccaacgcgttggatgcatagcttgagtattctatagtgtcacctaaatagcttggcgtaatcatggtcatagctgtttcctgtgtgaaattgttatccgctcacaattccacacaacatacgagccggaagcataaagtgtaaagcctggggtgcctaatgagtgagctaactcacattaattgcgttgcgctcactgcccgctttccagtcgggaaacctgtcgtgccagctgcattaatgaatcggccaacgcgcggggagaggcggtttgcgtattgggcgctcttccgcttcctcgctcactgactcgctgcgctcggtcgttcggctgcggcgagcggtatcagctcactcaaaggcggtaatacggttatccacagaatcaggggataacgcaggaaagaacatgtgagcaaaaggccagcaaaaggccaggaaccgtaaaaaggccgcgttgctggcgtttttccataggctccgcccccctgacgagcatcacaaaaatcgacgctcaagtcagaggtggcgaaacccgacaggactataaagataccaggcgtttccccctggaagctccctcgtgcgctctcctgttccgaccctgccgcttaccggatacctgtccgcctttctcccttcgggaagcgtggcgctttctcatagctcacgctgtaggtatctcagttcggtgtaggtcgttcgctccaagctgggctgtgtgcacgaaccccccgttcagcccgaccgctgcgccttatccggtaactatcgtcttgagtccaacccggtaagacacgacttatcgccactggcagcagccactggtaacaggattagcagagcgaggtatgtaggcggtgctacagagttcttgaagtggtggcctaactacggctacactagaagaacagtatttggtatctgcgctctgctgaagccagttaccttcggaaaaagagttggtagctcttgatccggcaaacaaaccaccgctggtagcggtggtttttttgtttgcaagcagcagattacgcgcagaaaaaaaggatctcaagaagatcctttgatcttttctacggggtctgacgctcagtggaacgaaaactcacgttaagggattttggtcatgagattatcaaaaaggatcttcacctagatccttttaaattaaaaatgaagttttaaatcaatctaaagtatatatgagtaaacttggtctgacagttaccaatgcttaatcagtgaggcacctatctcagcgatctgtctatttcgttcatccatagttgcctgactccccgtcgtgtagataactacgatacgggagggcttaccatctggccccagtgctgcaatgataccgcgagacccacgctcaccggctccagatttatcagcaataaaccagccagccggaagggccgagcgcagaagtggtcctgcaactttatccgcctccatccagtctattaattgttgccgggaagctagagtaagtagttcgccagttaatagtttgcgcaacgttgttgccattgctacaggcatcgtggtgtcacgctcgtcgtttggtatggcttcattcagctccggttcccaacgatcaaggcgagttacatgatcccccatgttgtgcaaaaaagcggttagctccttcggtcctccgatcgttgtcagaagtaagttggccgcagtgttatcactcatggttatggcagcactgcataattctcttactgtcatgccatccgtaagatgcttttctgtgactggtgagtactcaaccaagtcattctgagaatagtgtatgcggcgaccgagttgctcttgcccggcgtcaatacgggataataccgcgccacatagcagaactttaaaagtgctcatcattggaaaacgttcttcggggcgaaaactctcaaggatcttaccgctgttgagatccagttcgatgtaacccactcgtgcacccaactgatcttcagcatcttttactttcaccagcgtttctgggtgagcaaaaacaggaaggcaaaatgccgcaaaaaagggaataagggcgacacggaaatgttgaatactcatactcttcctttttcaatattattgaagcatttatcagggttattgtctcatgagcggatacatatttgaatgtatttagaaaaataaacaaataggggttccgcgcacatttccccgaaaagtgccacctgatgcggtgtgaaataccgcacagatgcgtaaggagaaaataccgcatcaggaaattgtaagcgttaatattttgttaaaattcgcgttaaatttttgttaaatcagctcattttttaaccaataggccgaaatcggcaaaatcccttataaatcaaaagaatagaccgagatagggttgagtgttgttccagtttggaacaagagtccactattaaagaacgtggactccaacgtcaaagggcgaaaaaccgtctatcagggcgatggcccactacgtgaaccatcaccctaatcaagttttttggggtcgaggtgccgtaaagcactaaatcggaaccctaaagggagcccccgatttagagcttgacggggaaagccggcgaacgtggcgagaaaggaagggaagaaagcgaaaggagcgggcgctagggcgctggcaagtgtagcggtcacgctgcgcgtaaccaccacacccgccgcgcttaatgcgccgctacagggcgcgtccattcgccattcaggctgcgcaactgttgggaagggcgatcggtgcgggcctcttcgctattacgccagctggcgaaagggggatgtgctgcaaggcgattaagttgggtaacgccagggttttcccagtcacgacgttgtaaaacgacggccagtgaattgtaatacgactcactatagggcgaattgggcccgacgtcgcatgctcccggccgccatggcggccgcgggaattcgattgaggcatgctaatacgactcactatagg

SEQ ID NO: 11 - RNA, 21 nt, artificial
  microRNA
uggaauguaaagaaguaugua

SEQ ID NO: 12 - RNA, 22 nt, artificial
  microRNA
uacaguacugugauaacugaag

SEQ ID NO: 13 - RNA, 23 nt, artificial
  microRNA
uggagugugacaaugguguuugu

SEQ ID NO: 14 - RNA, 22 nt, artificial
  microRNA
uuaaggcacgcggugaaugcca

SEQ ID NO: 15 - RNA, 23 nt, artificial
  microRNA
ucccugagacccuuuaaccugug

SEQ ID NO: 16 - RNA, 21 nt, artificial
  microRNA
ucguaccgugaguaauaaugc

SEQ ID NO: 17 - RNA, 22 nt, artificial
  microRNA
ucggauccgucugagcuuggcu

SEQ ID NO: 18 - RNA, 22 nt, artificial
  microRNA
ucacagugaaccggucucuuuc

SEQ ID NO: 19 - RNA, 22 nt, artificial
  microRNA
cagugcaauguuaaaagggcau

SEQ ID NO: 20 - RNA, 22 nt, artificial
  microRNA
uaacagucuacagccauggucg

SEQ ID NO: 21 - RNA, 22 nt, artificial
  microRNA
uugguccccuucaaccagcugu

SEQ ID NO: 22 - RNA, 21 nt, artificial
  microRNA
ugugacugguugaccagaggg

SEQ ID NO: 23 - RNA, 23 nt, artificial
  microRNA
uauggcuuuuuauuccuauguga

SEQ ID NO: 24 - RNA, 17 nt, artificial
  microRNA
agcugguguugugaauc

SEQ ID NO: 25 - RNA, 20 nt, artificial
  microRNA
cauaaaguagaaagcacuac

SEQ ID NO: 26 - RNA, 23 nt, artificial
  microRNA
uguaguguuuccuacuuuaugga

SEQ ID NO: 27 - RNA, 22 nt, artificial
  microRNA
ugagaugaagcacuguagcuca

SEQ ID NO: 28 - RNA, 24 nt, artificial
  microRNA
guccaguuuucccaggaaucccuu

SEQ ID NO: 29 - RNA, 22 nt, artificial
  microRNA
ucagugcacuacagaacuuugu

SEQ ID NO: 30 - RNA, 22 nt, artificial
  microRNA
uagcagcacauaaugguuugug

SEQ ID NO: 31 - RNA, 22 nt, artificial
  microRNA
ucucccaacccuuguaccagug

SEQ ID NO: 32 - RNA, 22 nt, artificial
  microRNA
acuagacugaagcuccuugagg

SEQ ID NO: 33 - RNA, 22 nt, artificial
  microRNA
ucagugcaugacagaacuuggg

SEQ ID NO: 34 - RNA, 20 nt, artificial
  microRNA
uugcauagucacaaaaguga

SEQ ID NO: 35 - RNA, 22 nt, artificial
  microRNA
uuaaugcuaaucgugauagggg

SEQ ID NO: 36 - RNA, 22 nt, artificial
  microRNA
uagcagcacguaaauauuggcg

SEQ ID NO: 37 - RNA, 24 nt, artificial
  microRNA
caaagugcuuacagugcagguagu

SEQ ID NO: 38 - RNA, 23 nt, artificial
  microRNA
aacauucaacgcugucggugagu

SEQ ID NO: 39 - RNA, 23 nt, artificial
  microRNA
uauggcacugguagaauucacug

SEQ ID NO: 40 - RNA, 22 nt, artificial
  microRNA
uaaggugcaucuagugcagaua

SEQ ID NO: 41 - RNA, 22 nt, artificial
  microRNA
uaaggugcaucuagugcaguua

SEQ ID NO: 42 - RNA, 21 nt, artificial
  microRNA
cugaccuaugaauugacagcc

SEQ ID NO: 43 - RNA, 22 nt, artificial
  microRNA
uguaacagcaacuccaugugga

SEQ ID NO: 44 - RNA, 21 nt, artificial
  microRNA
uagcagcacagaaauauuggc

SEQ ID NO: 45 - RNA, 23 nt, artificial
  microRNA
cccaguguucagacuaccuguuc

SEQ ID NO: 46 - RNA, 23 nt, artificial
  microRNA
ugugcaaaucuaugcaaaacuga

SEQ ID NO: 47 - RNA, 23 nt, artificial
  microRNA
ugugcaaauccaugcaaaacuga

SEQ ID NO: 48 - RNA, 22 nt, artificial
  microRNA
uucccuuugucauccuaugccu

SEQ ID NO: 49 - RNA, 22 nt, artificial
  microRNA
uucccuuugucauccuaugccu

SEQ ID NO: 50 - RNA, 22 nt, artificial
  microRNA
uggaauguaaggaagugugugg

SEQ ID NO: 51 - RNA, 22 nt, artificial
  microRNA
auaagacgagcaaaaagcuugu

SEQ ID NO: 52 - RNA, 21 nt, artificial
  microRNA
uaacagucuccagucacggcc

SEQ ID NO: 53 - RNA, 21 nt, artificial
  microRNA
augaccuaugaauugacagac

SEQ ID NO: 54 - RNA, 21 nt, artificial
  microRNA
augaccuaugaauugacagac

SEQ ID NO: 55 - RNA, 21 nt, artificial
  microRNA
uaaucucagcuggcaacugug

SEQ ID NO: 56 - RNA, 20 nt, artificial
  microRNA
ugauuguccaaacgcaauuc

SEQ ID NO: 57 - RNA, 23 nt, artificial
  microRNA
agcuacauugucugcuggguuuc

SEQ ID NO: 58 - RNA, 24 nt, artificial
  microRNA
agcuacaucuggcuacugggucuc

SEQ ID NO: 59 - RNA, 21 nt, artificial
  microRNA
ugucaguuugucaaauacccc

SEQ ID NO: 60 - RNA, 22 nt, artificial
  microRNA
uggcucaguucagcaggaacag

SEQ ID NO: 61 - RNA, 22 nt, artificial
  microRNA
cauugcacuugucucggucuga

SEQ ID NO: 62 - RNA, 22 nt, artificial
  microRNA
uguaaacauccuacacucagcu

SEQ ID NO: 63 - RNA, 23 nt, artificial
  microRNA
uguaaacauccuacacucucagc

SEQ ID NO: 64 - RNA, 21 nt, artificial
  microRNA
uauugcacauuacuaaguugc

SEQ ID NO: 65 - RNA, 22 nt, artificial
  microRNA
uuuguucguucggcucgcguga

SEQ ID NO: 66 - RNA, 22 nt, artificial
  microRNA
uggaagacuagugauuuuguug

SEQ ID NO: 67 - RNA, 23 nt, artificial
  microRNA
ucuuugguuaucuagcuguauga

SEQ ID NO: 68 - RNA, 22 nt, artificial
  microRNA
uucaacggguauuuauugagca

SEQ ID NO: 69 - RNA, 22 nt, artificial
  microRNA
cacccguagaaccgaccuugcg